European Patent Application EP 4 650 445 A1, published November 19, 2025. Title: ゲノムまたはメタゲノム解析のための内部標準核酸. Applicant: 国立研究開発法人産業技術総合研究所. Application JP. The sequence listing filed with the application follows.

SEQUENCE LISTING (23 sequences)

SEQ ID NO: 1 - protein, 105 aa, synthetic construct
  REGION 1..105: note = TIGR01079
  REGION 2..3: note = misc_feature - Xaa can be any naturally occurring amino acid
  SITE 7: note = misc_feature - Xaa can be any naturally occurring amino acid
  SITE 10: note = misc_feature - Xaa can be any naturally occurring amino acid
  SITE 12: note = misc_feature - Xaa can be any naturally occurring amino acid
  SITE 15: note = misc_feature - Xaa can be any naturally occurring amino acid
  SITE 18: note = misc_feature - Xaa can be any naturally occurring amino acid
  REGION 21..22: note = misc_feature - Xaa can be any naturally occurring amino acid
  SITE 24: note = misc_feature - Xaa can be any naturally occurring amino acid
  REGION 26..27: note = misc_feature - Xaa can be any naturally occurring amino acid
  REGION 29..34: note = misc_feature - Xaa can be any naturally occurring amino acid
  REGION 41..43: note = misc_feature - Xaa can be any naturally occurring amino acid
  REGION 46..47: note = misc_feature - Xaa can be any naturally occurring amino acid
  REGION 49..56: note = misc_feature - Xaa can be any naturally occurring amino acid
  REGION 58..62: note = misc_feature - Xaa can be any naturally occurring amino acid
  SITE 64: note = misc_feature - Xaa can be any naturally occurring amino acid
  REGION 67..68: note = misc_feature - Xaa can be any naturally occurring amino acid
  REGION 72..83: note = misc_feature - Xaa can be any naturally occurring amino acid
  REGION 85..86: note = misc_feature - Xaa can be any naturally occurring amino acid
  REGION 88..93: note = misc_feature - Xaa can be any naturally occurring amino acid
  SITE 95: note = misc_feature - Xaa can be any naturally occurring amino acid
  REGION 97..101: note = misc_feature - Xaa can be any naturally occurring amino acid
  REGION 103..104: note = misc_feature - Xaa can be any naturally occurring amino acid
MXXKIKXGDXVXVIXGKXKGXXGXVXXVXXXXXXVIVEGVXXXKKXXKXXXXXXXXGXXXXXEXPIXXSNVXXXXXXXXXXXXVXXRXXXXXXKXRXXXXXGXXI

SEQ ID NO: 2 - protein, 115 aa, synthetic construct
  REGION 1..115: note = TIGR01024
  REGION 2..4: note = misc_feature - Xaa can be any naturally occurring amino acid
  REGION 6..7: note = misc_feature - Xaa can be any naturally occurring amino acid
  REGION 9..20: note = misc_feature - Xaa can be any naturally occurring amino acid
  REGION 22..23: note = misc_feature - Xaa can be any naturally occurring amino acid
  REGION 25..26: note = misc_feature - Xaa can be any naturally occurring amino acid
  SITE 28: note = misc_feature - Xaa can be any naturally occurring amino acid
  REGION 30..32: note = misc_feature - Xaa can be any naturally occurring amino acid
  SITE 34: note = misc_feature - Xaa can be any naturally occurring amino acid
  REGION 37..39: note = misc_feature - Xaa can be any naturally occurring amino acid
  SITE 41: note = misc_feature - Xaa can be any naturally occurring amino acid
  SITE 43: note = misc_feature - Xaa can be any naturally occurring amino acid
  SITE 45: note = misc_feature - Xaa can be any naturally occurring amino acid
  SITE 47: note = misc_feature - Xaa can be any naturally occurring amino acid
  REGION 50..54: note = misc_feature - Xaa can be any naturally occurring amino acid
  REGION 56..61: note = misc_feature - Xaa can be any naturally occurring amino acid
  SITE 63: note = misc_feature - Xaa can be any naturally occurring amino acid
  REGION 65..67: note = misc_feature - Xaa can be any naturally occurring amino acid
  SITE 69: note = misc_feature - Xaa can be any naturally occurring amino acid
  SITE 74: note = misc_feature - Xaa can be any naturally occurring amino acid
  REGION 76..81: note = misc_feature - Xaa can be any naturally occurring amino acid
  REGION 83..84: note = misc_feature - Xaa can be any naturally occurring amino acid
  SITE 86: note = misc_feature - Xaa can be any naturally occurring amino acid
  REGION 88..90: note = misc_feature - Xaa can be any naturally occurring amino acid
  SITE 92: note = misc_feature - Xaa can be any naturally occurring amino acid
  SITE 94: note = misc_feature - Xaa can be any naturally occurring amino acid
  SITE 97: note = misc_feature - Xaa can be any naturally occurring amino acid
  SITE 99: note = misc_feature - Xaa can be any naturally occurring amino acid
  REGION 103..105: note = misc_feature - Xaa can be any naturally occurring amino acid
  REGION 108..109: note = misc_feature - Xaa can be any naturally occurring amino acid
  REGION 113..115: note = misc_feature - Xaa can be any naturally occurring amino acid
MXXXIXXLXXXXXXXXXXXXFXXGXXVXVXXXIXEGXXXRXQXFXGXVIXXXXXGXXXXXXVXKXXXGXGVERXFXXXXXXIXXIXVXXXGXVXRAXLXYLRXXXGKXXKIKXXX

SEQ ID NO: 3 - protein, 116 aa, synthetic construct
  REGION 1..116: note = TIGR00082
  REGION 4..6: note = misc_feature - Xaa can be any naturally occurring amino acid
  REGION 8..9: note = misc_feature - Xaa can be any naturally occurring amino acid
  REGION 12..14: note = misc_feature - Xaa can be any naturally occurring amino acid
  REGION 16..18: note = misc_feature - Xaa can be any naturally occurring amino acid
  REGION 20..22: note = misc_feature - Xaa can be any naturally occurring amino acid
  REGION 24..26: note = misc_feature - Xaa can be any naturally occurring amino acid
  SITE 28: note = misc_feature - Xaa can be any naturally occurring amino acid
  REGION 30..36: note = misc_feature - Xaa can be any naturally occurring amino acid
  REGION 38..39: note = misc_feature - Xaa can be any naturally occurring amino acid
  SITE 42: note = misc_feature - Xaa can be any naturally occurring amino acid
  SITE 44: note = misc_feature - Xaa can be any naturally occurring amino acid
  REGION 47..50: note = misc_feature - Xaa can be any naturally occurring amino acid
  REGION 54..55: note = misc_feature - Xaa can be any naturally occurring amino acid
  SITE 57: note = misc_feature - Xaa can be any naturally occurring amino acid
  REGION 59..65: note = misc_feature - Xaa can be any naturally occurring amino acid
  REGION 67..68: note = misc_feature - Xaa can be any naturally occurring amino acid
  REGION 70..71: note = misc_feature - Xaa can be any naturally occurring amino acid
  SITE 73: note = misc_feature - Xaa can be any naturally occurring amino acid
  REGION 77..79: note = misc_feature - Xaa can be any naturally occurring amino acid
  REGION 81..85: note = misc_feature - Xaa can be any naturally occurring amino acid
  REGION 87..89: note = misc_feature - Xaa can be any naturally occurring amino acid
  SITE 91: note = misc_feature - Xaa can be any naturally occurring amino acid
  SITE 93: note = misc_feature - Xaa can be any naturally occurring amino acid
  REGION 95..96: note = misc_feature - Xaa can be any naturally occurring amino acid
  SITE 98: note = misc_feature - Xaa can be any naturally occurring amino acid
  REGION 101..104: note = misc_feature - Xaa can be any naturally occurring amino acid
  REGION 107..108: note = misc_feature - Xaa can be any naturally occurring amino acid
  REGION 111..112: note = misc_feature - Xaa can be any naturally occurring amino acid
  REGION 114..116: note = misc_feature - Xaa can be any naturally occurring amino acid
MMAXXXRXXRVXXXIXXXIXXXLXXXIXDXXXXXXXVXXVEXSXDLXXXXVFVXXLXDXXXXXXXVXXLXXAXGFIXXXLXXXXXLXXXPXLXFXXDXSLXXXXRIXXLIXXLXXX

SEQ ID NO: 4 - protein, 299 aa, synthetic construct
  REGION 1..299: note = TIGR02027
  REGION 2..4: note = misc_feature - Xaa can be any naturally occurring amino acid
  REGION 6..8: note = misc_feature - Xaa can be any naturally occurring amino acid
  REGION 11..12: note = misc_feature - Xaa can be any naturally occurring amino acid
  SITE 14: note = misc_feature - Xaa can be any naturally occurring amino acid
  SITE 16: note = misc_feature - Xaa can be any naturally occurring amino acid
  REGION 20..21: note = misc_feature - Xaa can be any naturally occurring amino acid
  REGION 28..29: note = misc_feature - Xaa can be any naturally occurring amino acid
  SITE 31: note = misc_feature - Xaa can be any naturally occurring amino acid
  SITE 33: note = misc_feature - Xaa can be any naturally occurring amino acid
  REGION 36..39: note = misc_feature - Xaa can be any naturally occurring amino acid
  REGION 41..45: note = misc_feature - Xaa can be any naturally occurring amino acid
  REGION 48..51: note = misc_feature - Xaa can be any naturally occurring amino acid
  SITE 54: note = misc_feature - Xaa can be any naturally occurring amino acid
  REGION 58..59: note = misc_feature - Xaa can be any naturally occurring amino acid
  SITE 62: note = misc_feature - Xaa can be any naturally occurring amino acid
  SITE 66: note = misc_feature - Xaa can be any naturally occurring amino acid
  REGION 68..91: note = misc_feature - Xaa can be any naturally occurring amino acid
  REGION 93..101: note = misc_feature - Xaa can be any naturally occurring amino acid
  REGION 105..110: note = misc_feature - Xaa can be any naturally occurring amino acid
  REGION 112..113: note = misc_feature - Xaa can be any naturally occurring amino acid
  REGION 115..119: note = misc_feature - Xaa can be any naturally occurring amino acid
  SITE 121: note = misc_feature - Xaa can be any naturally occurring amino acid
  SITE 123: note = misc_feature - Xaa can be any naturally occurring amino acid
  SITE 125: note = misc_feature - Xaa can be any naturally occurring amino acid
  REGION 127..128: note = misc_feature - Xaa can be any naturally occurring amino acid
  SITE 130: note = misc_feature - Xaa can be any naturally occurring amino acid
  REGION 133..147: note = misc_feature - Xaa can be any naturally occurring amino acid
  SITE 149: note = misc_feature - Xaa can be any naturally occurring amino acid
  SITE 153: note = misc_feature - Xaa can be any naturally occurring amino acid
  SITE 155: note = misc_feature - Xaa can be any naturally occurring amino acid
  REGION 158..159: note = misc_feature - Xaa can be any naturally occurring amino acid
  SITE 161: note = misc_feature - Xaa can be any naturally occurring amino acid
  SITE 163: note = misc_feature - Xaa can be any naturally occurring amino acid
  REGION 165..175: note = misc_feature - Xaa can be any naturally occurring amino acid
  SITE 177: note = misc_feature - Xaa can be any naturally occurring amino acid
  SITE 179: note = misc_feature - Xaa can be any naturally occurring amino acid
  SITE 181: note = misc_feature - Xaa can be any naturally occurring amino acid
  SITE 183: note = misc_feature - Xaa can be any naturally occurring amino acid
  REGION 185..192: note = misc_feature - Xaa can be any naturally occurring amino acid
  REGION 195..196: note = misc_feature - Xaa can be any naturally occurring amino acid
  REGION 198..200: note = misc_feature - Xaa can be any naturally occurring amino acid
  REGION 202..204: note = misc_feature - Xaa can be any naturally occurring amino acid
  REGION 206..238: note = misc_feature - Xaa can be any naturally occurring amino acid
  REGION 240..241: note = misc_feature - Xaa can be any naturally occurring amino acid
  SITE 246: note = misc_feature - Xaa can be any naturally occurring amino acid
  REGION 248..249: note = misc_feature - Xaa can be any naturally occurring amino acid
  REGION 253..256: note = misc_feature - Xaa can be any naturally occurring amino acid
  REGION 258..259: note = misc_feature - Xaa can be any naturally occurring amino acid
  SITE 261: note = misc_feature - Xaa can be any naturally occurring amino acid
  REGION 265..270: note = misc_feature - Xaa can be any naturally occurring amino acid
  REGION 272..275: note = misc_feature - Xaa can be any naturally occurring amino acid
  SITE 279: note = misc_feature - Xaa can be any naturally occurring amino acid
  REGION 282..283: note = misc_feature - Xaa can be any naturally occurring amino acid
  REGION 286..288: note = misc_feature - Xaa can be any naturally occurring amino acid
  REGION 290..293: note = misc_feature - Xaa can be any naturally occurring amino acid
  SITE 295: note = misc_feature - Xaa can be any naturally occurring amino acid
  REGION 297..299: note = misc_feature - Xaa can be any naturally occurring amino acid
MXXXFXXXPLXXGXGXTLGXXLRRVLLXXIXGXAIXXXXIXXXXXEFXXXXGVXEDVXXIIXNLKXLXXXXXXXXXXXXXXXXXXXXXXXXAXXXXXXXXXVEVXXXXXXIXXLXXXXXLXIXLXVXXGXGYXXXXXXXXXXXXXXXIXVDAXFXPVXXVXYXVXXXXXXXXXXXDXLXLXIXTXXXXXXXXALXXAXXXLXXXLXXXXXXXXXXXXXXXXXXXXXXXXXXXXXXXXXIXXLDLSXRXXNCLXXXXIXXLXELVXXXXXXLXXXXNLGXKSXXEIXXXLXXXXLXLXXX

SEQ ID NO: 5 - protein, 330 aa, synthetic construct
  REGION 1..330: note = TIGR02729
  SITE 3: note = misc_feature - Xaa can be any naturally occurring amino acid
  REGION 5..9: note = misc_feature - Xaa can be any naturally occurring amino acid
  REGION 11..12: note = misc_feature - Xaa can be any naturally occurring amino acid
  SITE 14: note = misc_feature - Xaa can be any naturally occurring amino acid
  SITE 17: note = misc_feature - Xaa can be any naturally occurring amino acid
  REGION 19..24: note = misc_feature - Xaa can be any naturally occurring amino acid
  SITE 26: note = misc_feature - Xaa can be any naturally occurring amino acid
  REGION 28..30: note = misc_feature - Xaa can be any naturally occurring amino acid
  SITE 34: note = misc_feature - Xaa can be any naturally occurring amino acid
  SITE 37: note = misc_feature - Xaa can be any naturally occurring amino acid
  SITE 40: note = misc_feature - Xaa can be any naturally occurring amino acid
  SITE 43: note = misc_feature - Xaa can be any naturally occurring amino acid
  REGION 45..54: note = misc_feature - Xaa can be any naturally occurring amino acid
  REGION 56..65: note = misc_feature - Xaa can be any naturally occurring amino acid
  REGION 67..68: note = misc_feature - Xaa can be any naturally occurring amino acid
  REGION 70..71: note = misc_feature - Xaa can be any naturally occurring amino acid
  REGION 73..78: note = misc_feature - Xaa can be any naturally occurring amino acid
  REGION 80..86: note = misc_feature - Xaa can be any naturally occurring amino acid
  SITE 88: note = misc_feature - Xaa can be any naturally occurring amino acid
  SITE 91: note = misc_feature - Xaa can be any naturally occurring amino acid
  REGION 93..94: note = misc_feature - Xaa can be any naturally occurring amino acid
  REGION 96..118: note = misc_feature - Xaa can be any naturally occurring amino acid
  REGION 121..122: note = misc_feature - Xaa can be any naturally occurring amino acid
  SITE 124: note = misc_feature - Xaa can be any naturally occurring amino acid
  REGION 127..128: note = misc_feature - Xaa can be any naturally occurring amino acid
  REGION 130..136: note = misc_feature - Xaa can be any naturally occurring amino acid
  REGION 138..142: note = misc_feature - Xaa can be any naturally occurring amino acid
  REGION 144..150: note = misc_feature - Xaa can be any naturally occurring amino acid
  SITE 152: note = misc_feature - Xaa can be any naturally occurring amino acid
  SITE 154: note = misc_feature - Xaa can be any naturally occurring amino acid
  REGION 156..157: note = misc_feature - Xaa can be any naturally occurring amino acid
  REGION 166..169: note = misc_feature - Xaa can be any naturally occurring amino acid
  SITE 173: note = misc_feature - Xaa can be any naturally occurring amino acid
  REGION 176..184: note = misc_feature - Xaa can be any naturally occurring amino acid
  REGION 186..187: note = misc_feature - Xaa can be any naturally occurring amino acid
  SITE 189: note = misc_feature - Xaa can be any naturally occurring amino acid
  SITE 191: note = misc_feature - Xaa can be any naturally occurring amino acid
  REGION 193..194: note = misc_feature - Xaa can be any naturally occurring amino acid
  SITE 196: note = misc_feature - Xaa can be any naturally occurring amino acid
  REGION 199..210: note = misc_feature - Xaa can be any naturally occurring amino acid
  REGION 218..222: note = misc_feature - Xaa can be any naturally occurring amino acid
  SITE 224: note = misc_feature - Xaa can be any naturally occurring amino acid
  REGION 228..229: note = misc_feature - Xaa can be any naturally occurring amino acid
  SITE 232: note = misc_feature - Xaa can be any naturally occurring amino acid
  REGION 235..239: note = misc_feature - Xaa can be any naturally occurring amino acid
  REGION 241..242: note = misc_feature - Xaa can be any naturally occurring amino acid
  REGION 245..264: note = misc_feature - Xaa can be any naturally occurring amino acid
  REGION 266..267: note = misc_feature - Xaa can be any naturally occurring amino acid
  REGION 269..271: note = misc_feature - Xaa can be any naturally occurring amino acid
  REGION 273..282: note = misc_feature - Xaa can be any naturally occurring amino acid
  SITE 284: note = misc_feature - Xaa can be any naturally occurring amino acid
  REGION 286..330: note = misc_feature - Xaa can be any naturally occurring amino acid
MFXDXXXXXVXXGXGGXGXXXXXXEXYXXXGGPXGGXGGXGGXVXXXXXXXXXXLXXXXXXXXXXAXXGXXGXXXXXXGXXXXXXXIXVPXGXXVXXXXXXXXXXXXXXXXXXXXXXXGGXXGXGNXXFXXXXXXXPXXXXXGXXXXXXXLXLXLXXLADVGLVGXXXXGKSXLLXXXXXXXXXIXXYXFXTXXPXLGXXXXXXXXXXXXADIPGLIXXXXXGXGLGXXFLXHIXXXXXLXXLIXXXXXXXXXXXXXXXXXXXXLXXYXXXLXXXXXXXXXXKXDXXXXXXXXXXXXXXXXXXXXXXXXXXXXXXXXXXXXXXXXXXXXX

SEQ ID NO: 6 - protein, 271 aa, synthetic construct
  REGION 1..271: note = TIGR00436
  REGION 2..3: note = misc_feature - Xaa can be any naturally occurring amino acid
  REGION 9..10: note = misc_feature - Xaa can be any naturally occurring amino acid
  SITE 12: note = misc_feature - Xaa can be any naturally occurring amino acid
  SITE 20: note = misc_feature - Xaa can be any naturally occurring amino acid
  REGION 22..27: note = misc_feature - Xaa can be any naturally occurring amino acid
  SITE 29: note = misc_feature - Xaa can be any naturally occurring amino acid
  REGION 31..34: note = misc_feature - Xaa can be any naturally occurring amino acid
  REGION 37..39: note = misc_feature - Xaa can be any naturally occurring amino acid
  SITE 41: note = misc_feature - Xaa can be any naturally occurring amino acid
  REGION 43..49: note = misc_feature - Xaa can be any naturally occurring amino acid
  SITE 51: note = misc_feature - Xaa can be any naturally occurring amino acid
  REGION 60..62: note = misc_feature - Xaa can be any naturally occurring amino acid
  REGION 64..68: note = misc_feature - Xaa can be any naturally occurring amino acid
  SITE 71: note = misc_feature - Xaa can be any naturally occurring amino acid
  SITE 73: note = misc_feature - Xaa can be any naturally occurring amino acid
  REGION 75..76: note = misc_feature - Xaa can be any naturally occurring amino acid
  REGION 79..80: note = misc_feature - Xaa can be any naturally occurring amino acid
  REGION 89..96: note = misc_feature - Xaa can be any naturally occurring amino acid
  REGION 98..99: note = misc_feature - Xaa can be any naturally occurring amino acid
  REGION 101..103: note = misc_feature - Xaa can be any naturally occurring amino acid
  REGION 105..112: note = misc_feature - Xaa can be any naturally occurring amino acid
  REGION 114..141: note = misc_feature - Xaa can be any naturally occurring amino acid
  SITE 144: note = misc_feature - Xaa can be any naturally occurring amino acid
  REGION 146..163: note = misc_feature - Xaa can be any naturally occurring amino acid
  REGION 165..171: note = misc_feature - Xaa can be any naturally occurring amino acid
  SITE 173: note = misc_feature - Xaa can be any naturally occurring amino acid
  SITE 175: note = misc_feature - Xaa can be any naturally occurring amino acid
  SITE 177: note = misc_feature - Xaa can be any naturally occurring amino acid
  REGION 179..182: note = misc_feature - Xaa can be any naturally occurring amino acid
  SITE 184: note = misc_feature - Xaa can be any naturally occurring amino acid
  SITE 186: note = misc_feature - Xaa can be any naturally occurring amino acid
  SITE 188: note = misc_feature - Xaa can be any naturally occurring amino acid
  REGION 195..199: note = misc_feature - Xaa can be any naturally occurring amino acid
  SITE 204: note = misc_feature - Xaa can be any naturally occurring amino acid
  SITE 206: note = misc_feature - Xaa can be any naturally occurring amino acid
  SITE 208: note = misc_feature - Xaa can be any naturally occurring amino acid
  REGION 210..221: note = misc_feature - Xaa can be any naturally occurring amino acid
  REGION 223..225: note = misc_feature - Xaa can be any naturally occurring amino acid
  SITE 227: note = misc_feature - Xaa can be any naturally occurring amino acid
  SITE 229: note = misc_feature - Xaa can be any naturally occurring amino acid
  SITE 231: note = misc_feature - Xaa can be any naturally occurring amino acid
  SITE 235: note = misc_feature - Xaa can be any naturally occurring amino acid
  REGION 240..241: note = misc_feature - Xaa can be any naturally occurring amino acid
  REGION 243..244: note = misc_feature - Xaa can be any naturally occurring amino acid
  SITE 247: note = misc_feature - Xaa can be any naturally occurring amino acid
  REGION 250..252: note = misc_feature - Xaa can be any naturally occurring amino acid
  REGION 254..255: note = misc_feature - Xaa can be any naturally occurring amino acid
  REGION 257..263: note = misc_feature - Xaa can be any naturally occurring amino acid
  SITE 265: note = misc_feature - Xaa can be any naturally occurring amino acid
  SITE 267: note = misc_feature - Xaa can be any naturally occurring amino acid
  SITE 269: note = misc_feature - Xaa can be any naturally occurring amino acid
MXXVAILGXXNXGKSTLLNXLXXXXXXIXSXXXXTTXXXIXGXXXXXXXQXIFIDTPGLXXXKXXXXXLLXKXIXXALXXVDLILFVVXXXXXXXXDXXLXXXLXXXXXXXXLXXXXXXXXXXXXXXXXXXXXXXXXXXXXIVXIXXXXXXXXXXXXXXXXXXLXXXXXXXPXDXVXDXXXXFXIXEXIREKILXXXXXEIPYXVXVXIXXXXXXXXXXXXIXXXIXVXRXSQKXIIIGXXGXXIKXIGXXXRXXLXXXXXXXVXLXLXVK

SEQ ID NO: 7 - protein, 127 aa, synthetic construct
  REGION 1..127: note = TIGR01164
  REGION 2..3: note = misc_feature - Xaa can be any naturally occurring amino acid
  REGION 6..10: note = misc_feature - Xaa can be any naturally occurring amino acid
  REGION 12..18: note = misc_feature - Xaa can be any naturally occurring amino acid
  REGION 20..26: note = misc_feature - Xaa can be any naturally occurring amino acid
  SITE 28: note = misc_feature - Xaa can be any naturally occurring amino acid
  SITE 31: note = misc_feature - Xaa can be any naturally occurring amino acid
  SITE 33: note = misc_feature - Xaa can be any naturally occurring amino acid
  REGION 35..41: note = misc_feature - Xaa can be any naturally occurring amino acid
  REGION 43..46: note = misc_feature - Xaa can be any naturally occurring amino acid
  REGION 48..52: note = misc_feature - Xaa can be any naturally occurring amino acid
  SITE 55: note = misc_feature - Xaa can be any naturally occurring amino acid
  SITE 57: note = misc_feature - Xaa can be any naturally occurring amino acid
  REGION 59..63: note = misc_feature - Xaa can be any naturally occurring amino acid
  SITE 66: note = misc_feature - Xaa can be any naturally occurring amino acid
  REGION 69..76: note = misc_feature - Xaa can be any naturally occurring amino acid
  REGION 79..81: note = misc_feature - Xaa can be any naturally occurring amino acid
  SITE 85: note = misc_feature - Xaa can be any naturally occurring amino acid
  REGION 89..90: note = misc_feature - Xaa can be any naturally occurring amino acid
  SITE 92: note = misc_feature - Xaa can be any naturally occurring amino acid
  REGION 94..96: note = misc_feature - Xaa can be any naturally occurring amino acid
  REGION 98..99: note = misc_feature - Xaa can be any naturally occurring amino acid
  SITE 101: note = misc_feature - Xaa can be any naturally occurring amino acid
  SITE 107: note = misc_feature - Xaa can be any naturally occurring amino acid
  REGION 110..116: note = misc_feature - Xaa can be any naturally occurring amino acid
  REGION 119..120: note = misc_feature - Xaa can be any naturally occurring amino acid
  REGION 122..123: note = misc_feature - Xaa can be any naturally occurring amino acid
  SITE 127: note = misc_feature - Xaa can be any naturally occurring amino acid
MXXPKXXXXXKXXXXXXXGXXXXXXXVXFGXYXLXXXXXXXIXXXXIXXXXXALXRXVXXXXXLWXRIXXXXXXXXKPXXXRMGXGKGXXEXWXXXVXXGXVLFELXGVXXXXXXXALXXAXXKLPX

SEQ ID NO: 8 - protein, 190 aa, synthetic construct
  REGION 1..190: note = TIGR02432
  SITE 2: note = misc_feature - Xaa can be any naturally occurring amino acid
  SITE 11: note = misc_feature - Xaa can be any naturally occurring amino acid
  REGION 14..15: note = misc_feature - Xaa can be any naturally occurring amino acid
  REGION 18..19: note = misc_feature - Xaa can be any naturally occurring amino acid
  REGION 21..32: note = misc_feature - Xaa can be any naturally occurring amino acid
  SITE 35: note = misc_feature - Xaa can be any naturally occurring amino acid
  REGION 39..40: note = misc_feature - Xaa can be any naturally occurring amino acid
  REGION 42..43: note = misc_feature - Xaa can be any naturally occurring amino acid
  REGION 45..50: note = misc_feature - Xaa can be any naturally occurring amino acid
  REGION 52..83: note = misc_feature - Xaa can be any naturally occurring amino acid
  REGION 86..87: note = misc_feature - Xaa can be any naturally occurring amino acid
  REGION 90..91: note = misc_feature - Xaa can be any naturally occurring amino acid
  REGION 93..103: note = misc_feature - Xaa can be any naturally occurring amino acid
  SITE 110: note = misc_feature - Xaa can be any naturally occurring amino acid
  SITE 113: note = misc_feature - Xaa can be any naturally occurring amino acid
  REGION 119..120: note = misc_feature - Xaa can be any naturally occurring amino acid
  SITE 122: note = misc_feature - Xaa can be any naturally occurring amino acid
  REGION 125..128: note = misc_feature - Xaa can be any naturally occurring amino acid
  SITE 131: note = misc_feature - Xaa can be any naturally occurring amino acid
  REGION 134..144: note = misc_feature - Xaa can be any naturally occurring amino acid
  SITE 146: note = misc_feature - Xaa can be any naturally occurring amino acid
  REGION 151..153: note = misc_feature - Xaa can be any naturally occurring amino acid
  SITE 155: note = misc_feature - Xaa can be any naturally occurring amino acid
  REGION 158..165: note = misc_feature - Xaa can be any naturally occurring amino acid
  REGION 167..170: note = misc_feature - Xaa can be any naturally occurring amino acid
  SITE 172: note = misc_feature - Xaa can be any naturally occurring amino acid
  REGION 175..178: note = misc_feature - Xaa can be any naturally occurring amino acid
  SITE 180: note = misc_feature - Xaa can be any naturally occurring amino acid
  SITE 183: note = misc_feature - Xaa can be any naturally occurring amino acid
  REGION 186..187: note = misc_feature - Xaa can be any naturally occurring amino acid
MXLLVAVSGGXDSXXLLXXLXXXXXXXXXXXXAAXVDHXXRXXSXXXXXXVXXXXXXXXXXXXXXXXXXXXXXXXXXXXXXXXARXXRYXXLXXXXXXXXXXXILTAHHXDDXIETILXXLXRGXXXXGLXGLXXXXXXXXXXXIXRPLLXXXKXEIXXXXXXXXLXXXXDXTNXXXXYXRNXIRXXLLP

SEQ ID NO: 9 - protein, 166 aa, synthetic construct
  REGION 1..166: note = TIGR00168
  REGION 4..5: note = misc_feature - Xaa can be any naturally occurring amino acid
  REGION 7..9: note = misc_feature - Xaa can be any naturally occurring amino acid
  REGION 12..13: note = misc_feature - Xaa can be any naturally occurring amino acid
  REGION 15..17: note = misc_feature - Xaa can be any naturally occurring amino acid
  REGION 19..22: note = misc_feature - Xaa can be any naturally occurring amino acid
  REGION 24..27: note = misc_feature - Xaa can be any naturally occurring amino acid
  REGION 31..32: note = misc_feature - Xaa can be any naturally occurring amino acid
  REGION 34..37: note = misc_feature - Xaa can be any naturally occurring amino acid
  SITE 42: note = misc_feature - Xaa can be any naturally occurring amino acid
  REGION 45..49: note = misc_feature - Xaa can be any naturally occurring amino acid
  SITE 52: note = misc_feature - Xaa can be any naturally occurring amino acid
  SITE 61: note = misc_feature - Xaa can be any naturally occurring amino acid
  REGION 63..65: note = misc_feature - Xaa can be any naturally occurring amino acid
  REGION 67..68: note = misc_feature - Xaa can be any naturally occurring amino acid
  REGION 70..71: note = misc_feature - Xaa can be any naturally occurring amino acid
  SITE 74: note = misc_feature - Xaa can be any naturally occurring amino acid
  REGION 76..77: note = misc_feature - Xaa can be any naturally occurring amino acid
  SITE 79: note = misc_feature - Xaa can be any naturally occurring amino acid
  SITE 84: note = misc_feature - Xaa can be any naturally occurring amino acid
  REGION 86..88: note = misc_feature - Xaa can be any naturally occurring amino acid
  REGION 90..92: note = misc_feature - Xaa can be any naturally occurring amino acid
  REGION 94..96: note = misc_feature - Xaa can be any naturally occurring amino acid
  REGION 98..103: note = misc_feature - Xaa can be any naturally occurring amino acid
  REGION 106..107: note = misc_feature - Xaa can be any naturally occurring amino acid
  REGION 109..110: note = misc_feature - Xaa can be any naturally occurring amino acid
  REGION 113..114: note = misc_feature - Xaa can be any naturally occurring amino acid
  REGION 116..118: note = misc_feature - Xaa can be any naturally occurring amino acid
  REGION 121..126: note = misc_feature - Xaa can be any naturally occurring amino acid
  REGION 128..130: note = misc_feature - Xaa can be any naturally occurring amino acid
  REGION 133..134: note = misc_feature - Xaa can be any naturally occurring amino acid
  REGION 136..159: note = misc_feature - Xaa can be any naturally occurring amino acid
  SITE 162: note = misc_feature - Xaa can be any naturally occurring amino acid
  REGION 164..166: note = misc_feature - Xaa can be any naturally occurring amino acid
MINXXIXXXEVXXIXXXGXXXXIXXXXEALXXAXXXXLDLVXISXXXXXPVXKILDYGKYXYXXXKXXKXXKKXQXXIXVKEVXLXXXIXXXDXXXKXXXXXXFLXXGXXVKXXVXXXGRXXXXXXLXXXVLXXVXXXXXXXXXXXXXXXXXXXXXXXXLLXPXXX

SEQ ID NO: 10 - protein, 226 aa, synthetic construct
  REGION 1..226: note = TIGR01011
  SITE 2: note = misc_feature - Xaa can be any naturally occurring amino acid
  SITE 4: note = misc_feature - Xaa can be any naturally occurring amino acid
  REGION 6..7: note = misc_feature - Xaa can be any naturally occurring amino acid
  REGION 9..15: note = misc_feature - Xaa can be any naturally occurring amino acid
  REGION 17..23: note = misc_feature - Xaa can be any naturally occurring amino acid
  REGION 25..28: note = misc_feature - Xaa can be any naturally occurring amino acid
  REGION 31..33: note = misc_feature - Xaa can be any naturally occurring amino acid
  REGION 35..39: note = misc_feature - Xaa can be any naturally occurring amino acid
  SITE 41: note = misc_feature - Xaa can be any naturally occurring amino acid
  REGION 43..48: note = misc_feature - Xaa can be any naturally occurring amino acid
  REGION 50..55: note = misc_feature - Xaa can be any naturally occurring amino acid
  REGION 57..65: note = misc_feature - Xaa can be any naturally occurring amino acid
  REGION 73..78: note = misc_feature - Xaa can be any naturally occurring amino acid
  REGION 80..82: note = misc_feature - Xaa can be any naturally occurring amino acid
  REGION 84..89: note = misc_feature - Xaa can be any naturally occurring amino acid
  REGION 92..93: note = misc_feature - Xaa can be any naturally occurring amino acid
  SITE 99: note = misc_feature - Xaa can be any naturally occurring amino acid
  SITE 101: note = misc_feature - Xaa can be any naturally occurring amino acid
  REGION 103..104: note = misc_feature - Xaa can be any naturally occurring amino acid
  REGION 107..109: note = misc_feature - Xaa can be any naturally occurring amino acid
  REGION 111..112: note = misc_feature - Xaa can be any naturally occurring amino acid
  REGION 114..115: note = misc_feature - Xaa can be any naturally occurring amino acid
  REGION 117..129: note = misc_feature - Xaa can be any naturally occurring amino acid
  REGION 133..142: note = misc_feature - Xaa can be any naturally occurring amino acid
  REGION 144..146: note = misc_feature - Xaa can be any naturally occurring amino acid
  SITE 148: note = misc_feature - Xaa can be any naturally occurring amino acid
  REGION 151..152: note = misc_feature - Xaa can be any naturally occurring amino acid
  REGION 154..156: note = misc_feature - Xaa can be any naturally occurring amino acid
  REGION 158..159: note = misc_feature - Xaa can be any naturally occurring amino acid
  SITE 161: note = misc_feature - Xaa can be any naturally occurring amino acid
  SITE 163: note = misc_feature - Xaa can be any naturally occurring amino acid
  REGION 165..167: note = misc_feature - Xaa can be any naturally occurring amino acid
  REGION 169..170: note = misc_feature - Xaa can be any naturally occurring amino acid
  SITE 173: note = misc_feature - Xaa can be any naturally occurring amino acid
  REGION 176..177: note = misc_feature - Xaa can be any naturally occurring amino acid
  SITE 179: note = misc_feature - Xaa can be any naturally occurring amino acid
  REGION 185..186: note = misc_feature - Xaa can be any naturally occurring amino acid
  SITE 188: note = misc_feature - Xaa can be any naturally occurring amino acid
  REGION 190..191: note = misc_feature - Xaa can be any naturally occurring amino acid
  REGION 193..194: note = misc_feature - Xaa can be any naturally occurring amino acid
  REGION 197..198: note = misc_feature - Xaa can be any naturally occurring amino acid
  SITE 201: note = misc_feature - Xaa can be any naturally occurring amino acid
  REGION 203..210: note = misc_feature - Xaa can be any naturally occurring amino acid
  REGION 212..219: note = misc_feature - Xaa can be any naturally occurring amino acid
  REGION 221..226: note = misc_feature - Xaa can be any naturally occurring amino acid
MXVXLXXLXXXXXXXGXXXXXXXPXXXXFIXXXRXXXXXIXLXXXXXXLXXXXXXVXXXXXXXXXILFVGTKXXXXXXVXXXAXXXXXXYVXXRWLGGXLXNXXTIXXXIXXLXXLXXXXXXXXXXXXXKKEXXXXXXXXXXLXXXLXGIXXLXXXPXXLXVXDXXXEXXAVXEAXXLXIPVVAXXDXNXXPXXVDXXIPXNXXXXXXXXLXXXXXXXXVXXXXXX

SEQ ID NO: 11 - protein, 112 aa, synthetic construct
  REGION 1..112: note = TIGR00043
  REGION 2..3: note = misc_feature - Xaa can be any naturally occurring amino acid
  SITE 5: note = misc_feature - Xaa can be any naturally occurring amino acid
  REGION 7..9: note = misc_feature - Xaa can be any naturally occurring amino acid
  REGION 11..17: note = misc_feature - Xaa can be any naturally occurring amino acid
  REGION 19..20: note = misc_feature - Xaa can be any naturally occurring amino acid
  REGION 23..24: note = misc_feature - Xaa can be any naturally occurring amino acid
  REGION 26..27: note = misc_feature - Xaa can be any naturally occurring amino acid
  REGION 34..50: note = misc_feature - Xaa can be any naturally occurring amino acid
  SITE 54: note = misc_feature - Xaa can be any naturally occurring amino acid
  REGION 57..59: note = misc_feature - Xaa can be any naturally occurring amino acid
  REGION 61..63: note = misc_feature - Xaa can be any naturally occurring amino acid
  REGION 65..77: note = misc_feature - Xaa can be any naturally occurring amino acid
  REGION 79..80: note = misc_feature - Xaa can be any naturally occurring amino acid
  SITE 83: note = misc_feature - Xaa can be any naturally occurring amino acid
  SITE 87: note = misc_feature - Xaa can be any naturally occurring amino acid
  REGION 92..99: note = misc_feature - Xaa can be any naturally occurring amino acid
  REGION 101..103: note = misc_feature - Xaa can be any naturally occurring amino acid
  REGION 105..106: note = misc_feature - Xaa can be any naturally occurring amino acid
  REGION 109..112: note = misc_feature - Xaa can be any naturally occurring amino acid
MXXLXLXXXDXXXXXXXNXXYRXXDXXTDVLSFXXXXXXXXXXXXXXXXXGDLXISXXXVXXXAXXXXXXXXXXXXXLXXHGXLHLXGYDHXXXXXXXXMXXXEXXILXXXX

SEQ ID NO: 12 - protein, 142 aa, synthetic construct
  REGION 1..142: note = TIGR01066
  REGION 2..12: note = misc_feature - Xaa can be any naturally occurring amino acid
  SITE 14: note = misc_feature - Xaa can be any naturally occurring amino acid
  REGION 16..17: note = misc_feature - Xaa can be any naturally occurring amino acid
  REGION 21..24: note = misc_feature - Xaa can be any naturally occurring amino acid
  REGION 30..31: note = misc_feature - Xaa can be any naturally occurring amino acid
  REGION 34..35: note = misc_feature - Xaa can be any naturally occurring amino acid
  SITE 37: note = misc_feature - Xaa can be any naturally occurring amino acid
  SITE 40: note = misc_feature - Xaa can be any naturally occurring amino acid
  REGION 42..43: note = misc_feature - Xaa can be any naturally occurring amino acid
  SITE 45: note = misc_feature - Xaa can be any naturally occurring amino acid
  REGION 47..48: note = misc_feature - Xaa can be any naturally occurring amino acid
  SITE 50: note = misc_feature - Xaa can be any naturally occurring amino acid
  SITE 53: note = misc_feature - Xaa can be any naturally occurring amino acid
  REGION 60..61: note = misc_feature - Xaa can be any naturally occurring amino acid
  SITE 63: note = misc_feature - Xaa can be any naturally occurring amino acid
  SITE 65: note = misc_feature - Xaa can be any naturally occurring amino acid
  SITE 67: note = misc_feature - Xaa can be any naturally occurring amino acid
  REGION 69..71: note = misc_feature - Xaa can be any naturally occurring amino acid
  SITE 73: note = misc_feature - Xaa can be any naturally occurring amino acid
  REGION 75..77: note = misc_feature - Xaa can be any naturally occurring amino acid
  REGION 79..81: note = misc_feature - Xaa can be any naturally occurring amino acid
  REGION 83..91: note = misc_feature - Xaa can be any naturally occurring amino acid
  REGION 93..100: note = misc_feature - Xaa can be any naturally occurring amino acid
  REGION 102..103: note = misc_feature - Xaa can be any naturally occurring amino acid
  SITE 106: note = misc_feature - Xaa can be any naturally occurring amino acid
  SITE 108: note = misc_feature - Xaa can be any naturally occurring amino acid
  REGION 111..113: note = misc_feature - Xaa can be any naturally occurring amino acid
  REGION 115..121: note = misc_feature - Xaa can be any naturally occurring amino acid
  SITE 123: note = misc_feature - Xaa can be any naturally occurring amino acid
  SITE 126: note = misc_feature - Xaa can be any naturally occurring amino acid
  REGION 128..133: note = misc_feature - Xaa can be any naturally occurring amino acid
  REGION 135..136: note = misc_feature - Xaa can be any naturally occurring amino acid
  REGION 138..142: note = misc_feature - Xaa can be any naturally occurring amino acid
MXXXXXXXXXXXRXWXXVDAXXXXLGRLAXXVAXXLXGKXKXXYXPXXDXGDXVIVINAXXVXLXGXKXXXKXYXXXSXXXGXXXXXXXXXLXXXXXXXXLXXAVXGXLPXXXLXXXXXXXLXVYXGXXXXXXAXXPXXXXX

SEQ ID NO: 13 - protein, 113 aa, synthetic construct
  REGION 1..113: note = TIGR00059
  REGION 2..4: note = misc_feature - Xaa can be any naturally occurring amino acid
  REGION 6..7: note = misc_feature - Xaa can be any naturally occurring amino acid
  REGION 9..12: note = misc_feature - Xaa can be any naturally occurring amino acid
  REGION 14..15: note = misc_feature - Xaa can be any naturally occurring amino acid
  REGION 19..23: note = misc_feature - Xaa can be any naturally occurring amino acid
  REGION 26..29: note = misc_feature - Xaa can be any naturally occurring amino acid
  SITE 31: note = misc_feature - Xaa can be any naturally occurring amino acid
  REGION 34..35: note = misc_feature - Xaa can be any naturally occurring amino acid
  REGION 37..43: note = misc_feature - Xaa can be any naturally occurring amino acid
  SITE 46: note = misc_feature - Xaa can be any naturally occurring amino acid
  SITE 50: note = misc_feature - Xaa can be any naturally occurring amino acid
  REGION 53..59: note = misc_feature - Xaa can be any naturally occurring amino acid
  SITE 61: note = misc_feature - Xaa can be any naturally occurring amino acid
  REGION 63..65: note = misc_feature - Xaa can be any naturally occurring amino acid
  REGION 67..74: note = misc_feature - Xaa can be any naturally occurring amino acid
  REGION 77..78: note = misc_feature - Xaa can be any naturally occurring amino acid
  REGION 80..82: note = misc_feature - Xaa can be any naturally occurring amino acid
  REGION 84..85: note = misc_feature - Xaa can be any naturally occurring amino acid
  SITE 87: note = misc_feature - Xaa can be any naturally occurring amino acid
  REGION 96..98: note = misc_feature - Xaa can be any naturally occurring amino acid
  SITE 100: note = misc_feature - Xaa can be any naturally occurring amino acid
  SITE 103: note = misc_feature - Xaa can be any naturally occurring amino acid
  REGION 105..106: note = misc_feature - Xaa can be any naturally occurring amino acid
  SITE 108: note = misc_feature - Xaa can be any naturally occurring amino acid
MXXXKXXRXXXXRXXLLRXXXXXLLXXXXIXTTXXKXXXXXXXVEXLITXAKXXXXXXXRXVXXXLXXXXXXXXLFXXIXXXYXXRXGGYTRILKXXXRXGDXAXXAXLELVD

SEQ ID NO: 14 - protein, 294 aa, synthetic construct
  REGION 1..294: note = TIGR00116
  REGION 2..9: note = misc_feature - Xaa can be any naturally occurring amino acid
  SITE 12: note = misc_feature - Xaa can be any naturally occurring amino acid
  REGION 15..16: note = misc_feature - Xaa can be any naturally occurring amino acid
  SITE 18: note = misc_feature - Xaa can be any naturally occurring amino acid
  REGION 20..22: note = misc_feature - Xaa can be any naturally occurring amino acid
  SITE 26: note = misc_feature - Xaa can be any naturally occurring amino acid
  REGION 29..33: note = misc_feature - Xaa can be any naturally occurring amino acid
  REGION 36..37: note = misc_feature - Xaa can be any naturally occurring amino acid
  REGION 39..41: note = misc_feature - Xaa can be any naturally occurring amino acid
  REGION 44..45: note = misc_feature - Xaa can be any naturally occurring amino acid
  REGION 47..49: note = misc_feature - Xaa can be any naturally occurring amino acid
  SITE 51: note = misc_feature - Xaa can be any naturally occurring amino acid
  REGION 54..57: note = misc_feature - Xaa can be any naturally occurring amino acid
  SITE 59: note = misc_feature - Xaa can be any naturally occurring amino acid
  SITE 62: note = misc_feature - Xaa can be any naturally occurring amino acid
  REGION 64..73: note = misc_feature - Xaa can be any naturally occurring amino acid
  SITE 76: note = misc_feature - Xaa can be any naturally occurring amino acid
  REGION 78..80: note = misc_feature - Xaa can be any naturally occurring amino acid
  REGION 86..89: note = misc_feature - Xaa can be any naturally occurring amino acid
  REGION 91..92: note = misc_feature - Xaa can be any naturally occurring amino acid
  REGION 94..125: note = misc_feature - Xaa can be any naturally occurring amino acid
  REGION 127..130: note = misc_feature - Xaa can be any naturally occurring amino acid
  REGION 132..134: note = misc_feature - Xaa can be any naturally occurring amino acid
  SITE 136: note = misc_feature - Xaa can be any naturally occurring amino acid
  SITE 138: note = misc_feature - Xaa can be any naturally occurring amino acid
  REGION 143..152: note = misc_feature - Xaa can be any naturally occurring amino acid
  REGION 154..155: note = misc_feature - Xaa can be any naturally occurring amino acid
  SITE 157: note = misc_feature - Xaa can be any naturally occurring amino acid
  REGION 159..161: note = misc_feature - Xaa can be any naturally occurring amino acid
  REGION 168..180: note = misc_feature - Xaa can be any naturally occurring amino acid
  REGION 188..189: note = misc_feature - Xaa can be any naturally occurring amino acid
  REGION 191..192: note = misc_feature - Xaa can be any naturally occurring amino acid
  REGION 194..197: note = misc_feature - Xaa can be any naturally occurring amino acid
  REGION 199..202: note = misc_feature - Xaa can be any naturally occurring amino acid
  REGION 204..208: note = misc_feature - Xaa can be any naturally occurring amino acid
  REGION 210..219: note = misc_feature - Xaa can be any naturally occurring amino acid
  REGION 221..222: note = misc_feature - Xaa can be any naturally occurring amino acid
  REGION 224..227: note = misc_feature - Xaa can be any naturally occurring amino acid
  SITE 229: note = misc_feature - Xaa can be any naturally occurring amino acid
  SITE 233: note = misc_feature - Xaa can be any naturally occurring amino acid
  REGION 235..238: note = misc_feature - Xaa can be any naturally occurring amino acid
  SITE 240: note = misc_feature - Xaa can be any naturally occurring amino acid
  REGION 242..243: note = misc_feature - Xaa can be any naturally occurring amino acid
  SITE 245: note = misc_feature - Xaa can be any naturally occurring amino acid
  REGION 248..253: note = misc_feature - Xaa can be any naturally occurring amino acid
  REGION 255..257: note = misc_feature - Xaa can be any naturally occurring amino acid
  REGION 259..264: note = misc_feature - Xaa can be any naturally occurring amino acid
  REGION 266..267: note = misc_feature - Xaa can be any naturally occurring amino acid
  REGION 269..272: note = misc_feature - Xaa can be any naturally occurring amino acid
  SITE 278: note = misc_feature - Xaa can be any naturally occurring amino acid
  REGION 280..283: note = misc_feature - Xaa can be any naturally occurring amino acid
  REGION 285..286: note = misc_feature - Xaa can be any naturally occurring amino acid
  REGION 289..294: note = misc_feature - Xaa can be any naturally occurring amino acid
MXXXXXXXXVKXLRXXTXAXXXDCKXALXXXXXDLXXAXXXLRXXGXXXAXKKXXXXAXEGXVXXXXXXXXXXLVXIXXXTDFVAXXXXFXXLXXXXXXXXXXXXXXXXXXXXXXXXXXXXXXXXLXXXXAXXXEXIXVRRIXXXXXXXXXXIXXYXHXXXRIGVLVXXXXXXXXXXXXXLAMHVAAXXPXXLXXXXVXXXXVXXXXXIXXXXXXXXXXPXXIXXXXVXGRLXKXXXXIXLXXQXFVXXXXXXVXXXLXXXXXXVXXFXXXXVGEGIXKXXXXFXXEVXXXXXX

SEQ ID NO: 15 - protein, 149 aa, synthetic construct
  REGION 1..149: note = TIGR00158
  SITE 7: note = misc_feature - Xaa can be any naturally occurring amino acid
  SITE 9: note = misc_feature - Xaa can be any naturally occurring amino acid
  REGION 11..12: note = misc_feature - Xaa can be any naturally occurring amino acid
  REGION 15..16: note = misc_feature - Xaa can be any naturally occurring amino acid
  REGION 19..20: note = misc_feature - Xaa can be any naturally occurring amino acid
  SITE 24: note = misc_feature - Xaa can be any naturally occurring amino acid
  SITE 28: note = misc_feature - Xaa can be any naturally occurring amino acid
  SITE 33: note = misc_feature - Xaa can be any naturally occurring amino acid
  REGION 35..36: note = misc_feature - Xaa can be any naturally occurring amino acid
  REGION 38..40: note = misc_feature - Xaa can be any naturally occurring amino acid
  REGION 42..44: note = misc_feature - Xaa can be any naturally occurring amino acid
  REGION 46..77: note = misc_feature - Xaa can be any naturally occurring amino acid
  SITE 79: note = misc_feature - Xaa can be any naturally occurring amino acid
  REGION 81..82: note = misc_feature - Xaa can be any naturally occurring amino acid
  REGION 84..85: note = misc_feature - Xaa can be any naturally occurring amino acid
  SITE 87: note = misc_feature - Xaa can be any naturally occurring amino acid
  SITE 89: note = misc_feature - Xaa can be any naturally occurring amino acid
  SITE 93: note = misc_feature - Xaa can be any naturally occurring amino acid
  REGION 95..98: note = misc_feature - Xaa can be any naturally occurring amino acid
  SITE 100: note = misc_feature - Xaa can be any naturally occurring amino acid
  SITE 102: note = misc_feature - Xaa can be any naturally occurring amino acid
  REGION 104..109: note = misc_feature - Xaa can be any naturally occurring amino acid
  SITE 111: note = misc_feature - Xaa can be any naturally occurring amino acid
  REGION 113..114: note = misc_feature - Xaa can be any naturally occurring amino acid
  SITE 116: note = misc_feature - Xaa can be any naturally occurring amino acid
  REGION 118..125: note = misc_feature - Xaa can be any naturally occurring amino acid
  REGION 127..129: note = misc_feature - Xaa can be any naturally occurring amino acid
  SITE 131: note = misc_feature - Xaa can be any naturally occurring amino acid
  SITE 133: note = misc_feature - Xaa can be any naturally occurring amino acid
  REGION 135..136: note = misc_feature - Xaa can be any naturally occurring amino acid
  SITE 139: note = misc_feature - Xaa can be any naturally occurring amino acid
  SITE 141: note = misc_feature - Xaa can be any naturally occurring amino acid
  SITE 143: note = misc_feature - Xaa can be any naturally occurring amino acid
  SITE 145: note = misc_feature - Xaa can be any naturally occurring amino acid
  REGION 147..149: note = misc_feature - Xaa can be any naturally occurring amino acid
MMKVILXEXVXXLGXXGDXXEVKXGYAXNFLIXKXXAXXXTXXXIXXXXXXXXXXXXXXXXXXXXXXXXXXXXXXXXLXIXXKXXDXGXLFGXIXXXXIXDXVXXXXXXLXKXXIXLXXXXXXXXGXXXVXLXLXXEVXAXLXVXVXXX

SEQ ID NO: 16 - protein, 145 aa, synthetic construct
  REGION 1..145: note = TIGR01071
  SITE 2: note = misc_feature - Xaa can be any naturally occurring amino acid
  REGION 4..5: note = misc_feature - Xaa can be any naturally occurring amino acid
  REGION 7..18: note = misc_feature - Xaa can be any naturally occurring amino acid
  SITE 23: note = misc_feature - Xaa can be any naturally occurring amino acid
  SITE 27: note = misc_feature - Xaa can be any naturally occurring amino acid
  SITE 29: note = misc_feature - Xaa can be any naturally occurring amino acid
  SITE 31: note = misc_feature - Xaa can be any naturally occurring amino acid
  SITE 33: note = misc_feature - Xaa can be any naturally occurring amino acid
  SITE 35: note = misc_feature - Xaa can be any naturally occurring amino acid
  REGION 38..39: note = misc_feature - Xaa can be any naturally occurring amino acid
  REGION 42..49: note = misc_feature - Xaa can be any naturally occurring amino acid
  REGION 54..55: note = misc_feature - Xaa can be any naturally occurring amino acid
  REGION 58..59: note = misc_feature - Xaa can be any naturally occurring amino acid
  REGION 63..64: note = misc_feature - Xaa can be any naturally occurring amino acid
  REGION 66..76: note = misc_feature - Xaa can be any naturally occurring amino acid
  SITE 78: note = misc_feature - Xaa can be any naturally occurring amino acid
  REGION 80..91: note = misc_feature - Xaa can be any naturally occurring amino acid
  REGION 93..96: note = misc_feature - Xaa can be any naturally occurring amino acid
  REGION 98..102: note = misc_feature - Xaa can be any naturally occurring amino acid
  REGION 104..109: note = misc_feature - Xaa can be any naturally occurring amino acid
  REGION 114..145: note = misc_feature - Xaa can be any naturally occurring amino acid
MXLXXLXXXXXXXXXXXXVGRGXGSGXGXTXGXGXKGXXARXXXXXXXXFEGGXXPLXXRLPXXGXXXXXXXXXXXVXVXXXXXXXXXXXXVXXXXLXXXXXIXXXXXXVKVLXXXXXXXXXXXXXXXXXXXXXXXXXXXXXXXX

SEQ ID NO: 17 - DNA, 9932 bp, synthetic construct
  misc_feature 1..9932: note = seqHMM3501
  source 1..9932: mol_type = other DNA
gaatgcacagaatatcttacatcggtacaagaattcacagaatcgaatctcaacagaatcaaagcacgaattcatcaagaatcacttatcaagccttatctacagagaactttatcatcagattccatacagagttacaatcaggtattcacgtattcagacttactatacgcatttacagatcgtttcaaagaacaagaagcttctatacagtttctcacgaagttactttcgacaacttacaagaaagtcattctcacgattcaagatatacagaatgtactacaagattaagggaggagattcagttatagttatatacggtaagagtaagggtgaaattggtatagtaggaatagtagtctactactgtatcaaggtgattgtagaaggagtttcaagttcaaagaagtacgaaaagatcaacattcattcgtacgaatccggatcgtattcgtcatcagaacgaccaataaatacaagtaatgttagaatacgatcaaacatattacacgatacttacagagttgactatagaaacttatatcacatcagaaagagaagagttcagtcttacaagggaatatcgatttaatctgtcatattcacagctctattcctcaagaacttcacgtcgatggtttcgaacataatttcattgttccgaatatctcgaaacgacaatctcaacagtatattctattcgggttacacggtcacagttgaattcatcattaatgagggtgaaactgccagaatccagggattcaatggaatagttattagtattcgactctgtggaaacttctctgctatttcggtgcaaaagcaggtacaaggagacggtgtagagagagttttcaatctatactgctattacatagcttatattctggtgtcagaccaaggccttgttgaaagagctatactttcctaccttaggtcagttacaggtaagcaattaaagataaagaggctctattaagacatcagttactgttatatatacgaaggattccgtaccttaatgatggcatactacaagagataccagagagtaagagtcgacatagaattcagtattaagaagctgttatacacgtatattgttgatatcgtatatatcctgtaccaagtgtggacagttgaaagttcacgagatttgactctggaattcgtattcgtaacgttattatacgacgttatactggaaatatcagttgtattcggactgcacctggctataggtttcataatcagagaactaagtacgaaggtccgattgtactcaaagccaaagcttctattcgaaagtgacgtctcactgcatacagatctgagaattcaagtcttgataaatcagttaatctgtatttaatcgtacaagagatcaaatattacgagattcactggttacgtcatgatttacacattctatcaaagacctcttgtacatggaagaggttatacgcttggcttcagtttaaggagggtacttcttgactatattaatggatctgccataaagtaccatattataatacttacttacagcgaattcggcaacacagatggtgtatctgaagatgtagacaagataataatcaatctgaagtacttattctattactgtctcagtttctcgacgagtattatatacggaattatcaagtctggtaattctcagcattacgcaatacaggtatacgaattctcacagtcggtagaggtacaagcatacgacaagtcaattagagacttatattcgatatactatttgtctatctacttaacggttattcgaggctacggttatttccagtcgaatttacaggactctgcttcatcgatattatatcttattaaggttgatgcagaattcgatcctgtttacatagtttcctatagggtaatctgcaatccacatcagtatttatattacaaggattctcttatccttttcattagcacttatatatcagaaatcggtcagttcgcattggaacgcgcattattatatcttgatcaaagccttacttccatcgatcgattattattcagactttctcagagattcagatatccgaagtattacagaattcactacgcattatcttacttctcgaagcgttacatttcaaagcttgatttgtcatacagatactgcaattgtctttatcacgtacaaattgattctcttgaagaacttgttctattccaggatattcgtcttttccaaggatcaaatttgggtttcaagtcagagacggaaattttccgaaagttgagacgatattcgcttatcttgctacgtttataacttcgattcagaactacatacgcaagaattcgtttatctgctatgttccaagatgacgatttcgatctagtattatcgggcttcggtggatcaggtctcgaaatatccgttatcgaagaatacttcaaggaaggaggtccaagaggtggagttggaggcataggtggttcggtatacaaggatcaagtactatctattacagacctactcgtttattactgcaagagaatacagaaggcagtatacggttcgaatggatcacaggttattacggaaggtttctattaccgacaattatcaatagacgttccatcgggacatattgtgatcacgttccatatcaaggtatctctgttacaagtcaacaacgaatcaaaggatttacaagagaagcatggtggccacacaggacatggcaatgatatcttcaatacagctttactgtcagaccctttccagttatccagaggtattcactatcatcgttctacgttgatcttgcacttgcgttatttggcagatgttggacttgttggtagttcaagctgtggaaagtcactattattggattacaattacgatcaaggattaccaataacgatttatccattcaagaccttcataccaattttgggagttacaagacgcaaggtattacgatcattctgcaacgctgatatcccaggcttaattgtactttacatcgcaggatatggtttgggaaatcacttcttaattcacatcaacgcacttatacgattgctgttcttgatattcttatacgctgttcttacttacacgtatactcagtacatttatcagcatcggtatattctggaaacatattacgaaagtctcaagctacctttattccagaggattcattccaaggatgattacagcttcaatacaagaaaggttatactgcagattctatcaatcggcagattatacatcgtcattactttcaagaagctactcctgtctttacagaagcatcagatcagacaagaattctcagatacaaactgttaatgtttacttcaggattcagtaccagtatatcaattcgcaataatgacgagtgttgcaatattgggctctataaatcaaggtaagagtacgttacttaatctccttgcattattatcgcatttcattttaagtacaaggattaccacaacatatttcacaatttcgggtatattcgagttccttcgattccaaactatcttcattgatactccaggattgtatcgtttcaagttccaagcatcgattttacttccaaagcatattcaaagagctctttcgttcgtcgatttgatcttattcgtagtaatacttactgtatacaagtcacgtgattcagtattatacctatcgttaattactgtatcgtcttacataccactctatcgagaacatacgatcttattccagatcaggagcttcacaaacttctggaactcaatattcagtcaaatcggtcaattacacattgttttaataaagatacagaaggactaccgtatactcaaggacatttatctcgacagaacaatcttactgtatattcgtataccaattccagtagatacggttcaggatttacacaagattttcaagatttacgaatacataagggaaaagattttgattatcacagatcgtgaaataccgtattcagttccagtatacatacgattaccaagtttattccggacacgatctatttatatagatatccgaatatctgttatcagaagctcccaaaagtctattataatcggatatctaggacgaaagatcaagtacatcggaaagctcgttagatcgattttaaagtacatatcaaacgaagctgtatatctttgtttagttgttaagtaactattctggatccatttatcgatcgaagtatccatttcagttatgtctcacccaaagcagatacagtctgtaaagaatcgaaatatctgtctcactggcagttcacgcaatattacaacagtaagattcggttcgtatcctttaccagacttattcactgtacagatttcgctattacagatcgctatccaaagattcgcactgatcaggtcggtcatcttctgtggcaccttgtggaagcggatagaagtcgaaagtctatatacaaagaagccgtcagatttcagaatgggttccggaaagggcctacgagaaatctggtacagagatgtccggattggcttcgttcttttcgaattatctggtgtatatcacggtcatttatactacgcactttctgcagcgaagaataagctcccatcttaaatttcgaagtctcgagtcaagaagcatctgccaatttattcaatgtatcttttggtagcggttagcggtggtatagattcacactacttgctgaagtcgcttaatatatccacaaagttctcgcatttacagaagtcggcagctcgtgtagaccatacttcgcgcattaccagcttatccagtacacttatagtaaaggctttcctatattcggatacagatacacaagaacaaatctctggattcattcgagaacttcaagcttctatacacagaatacgggaaatttcggccagaacgaatagatattactctttgattcgcattaccagattatactggatatactgtatacttactgctcaccaccgagatgattcaatagaaacaatattagtttccctttatcggggttacagctctacaggccttcaaggattagcacatcaaagtttacgtacatctatccatcgtataatcagaccacttttgttcgttcgtaagctagaaataatatcagttcttcagaatatacgtcttcagttccaaggagatataacgaatctggaaacaaagtattcaagaaatcagataaggtatccacttttgccataagacaaggttctcaatctgtacaagaagttacaaccgtacttcatgataaatagaggaattattatacgagaagttcaaagaatttacgccataggcttacattattacatcaagtcattctccgaggctttgcgaatcgctaagttccagatccttgacttagtcttaatttcgtcagatcagacatatccagttcgcaagatattagattatggaaagtatctatacagaatcttcaagatacctaagaatcgtaagaagtaccagctgttcatatccgtaaaggaagtcaagttgcgatatataatagaatctacagatttcatccgcaagatatccgaaagtattacattcctacacttcggctcgcaagttaagagtatagtctcagatcgtggaagactattcgtacatcaagcattacactatacggttttgtctacagtcacaagaaagctatctttaccaacaggagttatcatatcgttcctcagtatcattctcaagggtccagtattacttcttaaccctgtttacgcataaaagtcttcgacttatcgattacaagaaagtctacgaaacgaaatgagtgtacaattgctattattaaggagtactcttcgaaagttcggacggaagaatttactacagacacctaatcagagttacttcatacacagtatccgccatcggatctatatcatctacttattactgggaaactcaacattacatcagattattactgcggtcttcttctgttacggaatactgttatcaatacttttcgttggtacgaagtcagcttcatactgttctgtgtcttacgcagcgcaaagagtctgctcactttatgtcatatcgagatggctcggcggatctttgacaaatatcatcacaataaaggacttcatatcgaacttgcaaactttggagaagttcatctgttcctatcatatcgagcagaacataaagaaggaatcaatatacgttcgatctcaaggtccatacttaacaagatacttaataggaatacaagatcttcagttacagccgcttatattaaacgtgatcgacaagttaccagaacaggatgcagtaagtgaagcttcactgttattcattcctgtagtggctctattcgattccaacgagcaacctatcaacgtagatatacgtataccgtctaatacatcgatatactcaaccgaaatcttaatttcaaaggcatcttatctgttagtcaaggttcaacgtattatttaatggaatcaaattctgtcagcttattcagcaatattctcgagaatgattcgattgtacctcattcaaacagataacttcaagctacagttccaaaatgctcaatacaggcaaggagatcaaagaacagatgtactttctttcatatacgagttccatctattccaggcttcgattatacagcagaattactgtggagatcttacaataagctcaattcaggtctacaatttcgcattatcttacaagaaggtattcaaggtcctttccaatattttatatcatcacggtacattacacttgacaggttatgatcattctttcagttctacaaacgatttcatgttcgctgttgaaattactatactaagatatcaacaataacattctaccagaagtactcttcgtactatactgtacatattcatgatactggaatatcagctgtcgaagtatcaattaagaacttggcgcagtgtggatgctcaaggatatttattaggtagattagctcgcttcgttgcttccacattgataggaaagattaagttatattactcaccacagaatgataagggagatcaggtaatagtcataaatgctacttctgtgttcttattaggagttaagacgaaggcaaagatatacatatctggatcttactgtcatggatcagacttccgttcattacttcgattcttgctcgaaattccagttctaccaaagcttattcgagcggttaatggagtgcttcctaatacgtctttgtatatcgaattcacataccgtttgatcgtttacacaggtttatcattcgaatctctagctattcttccagacgaagtattatcataacgttatctgttacgtatttcttcggatcaaatcaagtcaaagatgagattcacaaagatcgtcagaatacaatcagtcaggttcagattacttagacttctgcacaaggttctacttgctcatattcggattctaacgacaaacaacaagtacgacatcgatctatctgtagtagagtatcttataacatatgcaaagataccagacttcttcgttacaaggtatgtacaaagtttcttatctggaactctttcgtatctgttacttttccaagtcatatctgcagattaccacgtcagattcggtggatatacaaggatattaaagtcgttacggaggtatggtgactcagcacaaacagcgatccttgagcttgtcgattaagttctacaaatttcggcatatcctcgaacaagtctttatattatgacgaattcggctatacagaactctgtaaagattttgagaactgttacgtacgcgaaggtacacgattgtaagagtgccttaaaggtatcacaagttgatcttgatcatgcaagtatcttacttaggttcgaaggagatcatcaagcgacgaagaagtcatatacggaagcactagaaggctcagtatactgtttccaatcgaacaagacaagttatttggtttgtattttctggataactgacttcgttgcctcaaagaagggtttcacaacgttaaagcaagatttctggacatcagaattccttcatacaggtattacgattcctatacggaatcattcgatattatcggtcatcattcagattatctgcctcgaatctctcttagctcttcgcaaggagttcatccaagttagaagaatttattcaagacagttcgctttattcatcaagattgtcttctactaccatcgtattcgcagaattggcgtattggtcattcaccattacggattcaagtatcatttcacaaggactttagcgatgcacgtcgctgcgctataccctcaacagttgaccgatattcgagtatcattccacaaggtatatacactttcgagtatatcattctgtctactatcgagcgttatcaatccgtactcaattttcaccgatattgtttgcggaagattgtataagttccagattcttatcttactgaggctacagatattcgtcgttatacaacgcacattcgttataccgaagcttttacgtatcaacacttcagtgattcttttccagtatacgacggtaggagagggaatagttaagaatcacaagaatttctcgcaagaagtaagcttatcgtacaaggaataatcatcaacgtctttctcaagtcaacaggaattacagttatctatgatgaaggtgatccttgcagaagtagtgtcgagattgggaagtataggcgatacagtcgaagtcaagtatggttatgccattaacttcctcataaataaggctactgcgccgttatatacatatcgcattattgaaatcagaatccttacagagattattacgaacacattacgacgaagtatatctgtacaactctgttacgaatacttccttctgcaaattcagcttctttatatttcgtacaagcaagatgatcagggatacctgttcggttctattaggatcattattataccagacaaggtttattcaagcgaatcagttctgcgtaagatatctataatattgaggatcttcatatcgatctacaagggaattacgttcgtgagtttaacattgatttacgaagtgagcgctattcttgaggttcatgtacgagtactttaaatcgtcatattacatcacgattacatacagtcatcgtcttacatgtatttgcttatcttgcagttactctgtcaatcgttacgtttattcacggaagtaggtagaggcctgggctcaggtatcggaacaacaagcggtgttggttacaagggctacaaggcgagatctcatcaacgttatatctgtatcttcgagggaggaaatcgaccacttatcaagagattacctctgtctggatcgtatatccgagaaggtttattccaagttcttgtaggagtaattactcgaggtttatatcgtatttcgttactttcggtttcattacagacccttcatttactattctcgattacaacatcgttcagtacagtaaaggtgctattattcgaacatatcgtccaagaaactcgctattacgttatattctgcttacatcagctttcagtatcacatattccgattatttctctgcttatctaaactgtatattccatacgacaagattcagtttcaaattacgaaggtctactatttcacgagtcagaattctatatcgaaagcatttctcagtattccagtcttacagctttatttcatctgtcttctgttcaagaagttacatcgcaactttatactgcaaggaacaatctatacacatcgttcttatcgaaattacacgctcaagtatatcacaaaccgatttctgttactattcctacagcgtatattacaaacgacattccagaagattgcattc

SEQ ID NO: 18 - DNA, 9932 bp, synthetic construct
  misc_feature 1..9932: note = seqHMM5001
  source 1..9932: mol_type = other DNA
gaatgccaccgaagtacaggctcaatcgcgaccaattcataccgatcttcgtactccactcgacatccgctacctatatcggagattcaactccggcttcatactgtccgcaagtttacccgcatttacccaagcgagacgttatccgactcgatcatctcacagtcactccaccgagacagaatacacgaggactacgaatctgtcagcttccctctgtcacttacatcccggaacttattctcgggactcggaactttcagatccggccaagattatgcgcatcaagattaagttcggagatcgcgtcggcgtgatcgtcggcaagtctaagggtatcagtggtgaggtcgtcagtgtccactcagtcagagaagacgtcattgtggaaggcgtccggcacgaaaagaagcttcaaaaggctacaggcctttctgtcccgaagggagatacgaagaatccagaacaacctatctcggtatcaaacgtgatattcatcggcatctcacagcaacttccaacgcacgttaagtcacgctcctcaacgaacccttacaagggacgtttccataccagagcaggtgcagcaatttaattctctgtcgacatacagggtcgtcatccaggaccattcctcatggtctcgaagattgcactgctccctgtcagcgaaagttattcacgcctacctcacgtattcttcggtggtctacgtgtgttcgttcgcgaagtaatccacgaaggtagagtacctcgcaatcagtacttccgcggtctggttattaagagcgtacaaataggacaaccaagccatacggaagttcgaaagacacttcacggccgaggcgtggaacgcggtttcaccacgaagggatcgttcattaagagtatttccgtctggtatcggggcagtgttacgcgagcaacgctaggttacttgcgtacacgcacaggtaagcatccaaagatcaagagtcgagagtaactacgagacagctggaacacttacacgcaagcagtacatcgaatgatggcgtgcatctaccgcctgcgacgcgtatattcgcttattgctggatctattgtacgtcctctaaccgtctacatcatcgatttccgatctacgacatacgaggttcaattcgtagaatcttccgccgatcttacctgtgcgccggtcttcgtggtctacctgttcgacacactacatcaggacagacgcgttttcggtttaaagttcgcaacaggattcatccggagaatcctccgtataccaaacagcctcttcggaccaccataccttgacttcatacgagatcggtctctgcacggagttccacgtattaactcactgatctgcctcctgagatactcataaattccacatcatcaaggcttcggcacacttcatttccggtacatggaaacctcattctctcctcagccgctcaatctgggttctggagttacccttggtctcgtcttgcgccgcgttcttttgagaggaattttaggtgacgcgattattcgtctcaatatttccgaggagttctgtgagttcacagtcttcggaggtgtttcagaagatgtacacagaatcatcggcaacctcaagttcctgaccgcttccaggtcacacgtccatcggaagaactatatcgactcgagtctcctacctggacagaagcatctcgccatactccaaggtccgtcagtccgacaagttgaagtccgaaatctgtcagctggtattaacccgctcgatttcgacaactctctgctcatcaccttatccgtgccgagtggctcaggctacagtctcgagttccaactgcggcgtcatctacacaagcgatactcaattagggtggatgcggagttctcacctgttcggagcgtttcctacactgtgttcaagtcaggtacagtacctaagcgcaattcggattcgttgaggcttccaattgaaacgtatcacggatcaaccatcaccgatgctttacatctcgcaagaacactgctgcgaagacgtcttaagcgttcgtaccacgacaatcctatatcgtaccctgctgtcacatctcggagcacactttcgcttatcgttcgtccaacatacctcacagcggtcacaattcgtctactggacctctccttccgtctggctaattgcctggactgctattccatcaatacattgtgtgaattagtctcagtccagagcatcaacctgttccagactactaatctgggtgttaagagccaatacgaaatcgactcgaatttatccagagctattctgcgcttaacggatacctaagttcagtatcgacgagaagtacggcggatatctctgcagaagatgttcgcggacgacattacgaccgacgtcgtctcaggtattggtggctgtggcttcatccctgccacacgagaaaactattacgaggacggaggcccagaaggtggttctggtggccggggaggagaagtaactccacagatccacacggttatatccgcactcgtctatccaaactcgttccgggtccttcaagcggctcagggcctaccgggaaggctttcggttctcatcggcgagaggcataccaatcgtactatctcggtccctgttggcacgaccgtgacttcgtacatcaggcagacgagacagattcacacacaggcgttcactacactcggaaagcgtactacaggtggtcagcgaggtaccggcaatcatttcttccgattcacggtattctgggtaccgcgagacggattcacgggttatactccgcaatcgacatctctcggcctttatcttacaattcttgcggatgtgggtcttgtgggcgccatttccagtggcaagtcggtcctgttaaggcgattatcgccagaggatttcggtatccgagcctactacttcattacagcatccccgaccctgggtcgtccgacattcaccgaaattcgcaactccttcgttgccgatattccgggtctgattatctcacgaagctgcggttacggactgggcctacatttccttggtcatattacaggcagactttcgctttcaacactgattctcacgttcaccagtccgagtacacgttcaacattcccgggaggatactgtcagttcgcactggcagattacaactacggactcaactgggattacgtctccaccagtttcgaaaaggcagatatcgtcacatcgacggtacactcttcgccattcacgggaactgtacttcaccacgtcgttctctcaaggacgtacagctggttcacctacctgggactatcggatttcatcgcactcgtacgcatccaatcgtactaaatcagagagcaactctcgagaccgatctcatacttcctctgcatgcctcgtgtcgcgattctaggtacagataatctcggcaagtcgactctgctgaacgagctggatttccaacatcctggaatttgttccgcttcaggatcaacgacgacgctactaattatcggagtatctcagccttacaagagccagctaattttcattgacaccccgggactgctctcaaacaagcactcaacgctcgagctgctgcctaagtcaattccagatgctttgcaggaggtagatctgatactgttcgttgtaccagtctctttcgactggcacctggattacgttcttacagcgttactaagactcgaccagggatactctcggctgcacacgcttacaataccggagaccaggaatctcggttactgtacacgctcttacagtcaggctaccaaggcaaccgactatcgaattgtggacattcagtcacgcaattctctctggacataccacactgcgatcacgtactgtccgaagttaatcggttcaatccgacaacagcctagtgactccgtaacggatccactgtcagagttccgaatccctgaagccattcgtgaaaagattctggcactacacttctgcgaaattccgtacagtgtgcatgtgcagatcgaaatcggttcaacgtctgccgtcaaggtattcactatctgcaaggcgatcatcgtacctcgccacagtcaaaagttcatcatcatcggctctgctggaatcagaattaaggttatcggtcgcaatcaacgtccgttcctgaagagctcacttatttcccgcgtgttccttggattatacgtcaagtaaatcaagatccgtctgttacacgcccgattactcaaggcagagatgtgtactccgaaggtcggagactggtataaggaaacggatttccggttacatggcgcgagagcgacatacgcaaatgtgattttcggtgtataccgattggcgatatacaccgtactcaacataggaaattcccgcatttccgaagaacgtacagctttgctccgtaccgttgtaccttgcgccattctgtggccgcgtatcatacctatcacgaggagccaacgaaagccggcaagtcagcgcatgggtcttggtaagggctgtattgaatcttggatcaagtcagtggagctgggtagcgttctgttcgagttggatggtgtgctactgcagggatacggaacagctcttacagccgctaagcaaaagctgccagtttaaacgaagtctataccacgagcttctctcttcgctcagagctacatgcgtcttcttgtcgctgtaagcggtggtctggacagcggaggtctgctcactcctctgacgagggaagcacttccattcgtacgaaggtcgtatgcagcgcgcgttgaccaccaccaccgtgttaccagcggacaatcgcaagccttcgtggatctcacgagattacaggctgcgatcgcaagaaggaaggtcgttcgaagataccaggctcttccacgaccttcttcaacgactgtagaaatcgaggcacgtgtcgtccgctactcagcactgtacatacagggacacccttcctcgcacaagtacattctgacggcgcatcatcaagacgaccgcattgaaacaatcttaattcgactgcatcgcggtcgtcgaggacgtggactgggaggtttatcgaacgaagcatccggctcaacccaagtcctcatctctcgtccgctcctaggtacccgaaagactgaaatacaaatcttcaccgacaacacgctcctgagtacctaccaggacttcacaaatacgatcaggcactactaccgtaaccgaatccgcgatctcctgctcccttaatcagtacagcacacggttacgaacgttcataccgaggcgaatatgattaactcttcaatcaaggatcctgaagtaggacgaatagagggattcggtcttcgtcttcaaatccttcggaagacggaagcgctgtacttcgcacgaaccattccacttgacttagtgcggatctcgtatcaaggtaacgttcctgtgagtaagatactggattacggcaagtatctatatactggaaacaagtcgcgaaagacgtcgaagaagttccagcaactaatcctggttaaggaagtgcaactgatacttcgtatcctgtcagctgaccgcacaagcaagctcgttctccaagacgtattcctcgtcgttggtcaacttgtgaagagtcgagtacgcttatcaggtcgaaccgcatcgattacgaaccttaacccagtcgttctggtcatcgtgatccacacagttcgttcgagctctctatctgtcaggcatacctccatctgttcagagtaccctactaccctgcttttggccccgtctgcacattaattcctcgaacttcggtcagaccgaccatcaaccgatttcgaaatgattgtgtacctagtcacgctgttacgcgtatatcgagatcacggtcagtacgagagctcgggttccccgtcgttatccagtttcatttcattcgcacgcccgttacggatcttcattagcctgcatcactgggagtcgggattgcacaggatatctcatcaggtctcaactgcccgctgttactgcaaccacattctcttcgttggcacaaaggcgaggaacctctacttagtgtactactccgcaattctcgtaccgcctacgtacgtctcgttccgttggctcggcggatacttaccgaatcggataacgattgctcaaagtattggatcactggcacgcctgcacgaaatacacgctttacatcggagtcacagctcccaaaagaaggagaagtcccgaacaataccgaagccgaggttcctgtcggatatattaggcggaatcttccgtttgggccagataccggcactactcgacgtaagagatgatcaagccgagttcgttgctgtgtctgaagcatcttccctgatcatcccagtagtagcggctatcgatcagaatctcagcccgatcgaggttgacagttcgattcctcagaacaggcacagttacaccggttactaccttcactgcatacgccaaccgacatatgtgtacaaccaacaaactgcttaacagccagcacttcattctgcggaattacactgtcagacgctcatgagagtcctgcagctgccatatcaagattcagccggtaccaagaacataaatcgagcttatcgccgaaccgatcgcaggacagatgtgttgtccttcatttctccgtacgtaccgagactccatccagattatcggaacgataccgtaggcgatttaccaatctcgaatatacgagtgtcgagtcgcgcactacctcctagagaggatcatatctcgaacaggacactccttgagagccacggaagcttacatcttcgtggttatgatcattctatcgcgcatcacgtattccaaatggttcttccagagctttcgattctggagcatttctgttaaatccagaagcgatacgtcggaatctgggacaactaccaacgtatgtcctacaaggcaggcctatcatccaagcatcgccgtttatggcaagctgtagatgccggacaactacgtctgggacgactggcgccatcggttgcgtctcgtttaatcggcaagcacaagtatcagtatcggccgtcaggcgattcgggcgatccagtgattgttatcaacgctagtaccgtgcgattatcaggtacgaagagggactgtaagcgttatgagaacactagttccgaagtcggtactggaagtctccgagaggtttcattcttattacgaccaatcccgttcgcacgtttgacatacgcggtgcatggaatgttacctgttccaggattgacatactcgaccctacaggtcctgcacgtgtacgagggcaattatcgccgactcctagctgttcagccagttcgacttctcctttaacgcttacgagcaaccattcggtcaaagaggttcccgttccatatgatctgccctaaggccttacggagagctggaagtcgtgacaatctgctgcggcggttcctcttccgactgttgactgcgttcaagataggcactacgcatcgaaagaggtctgtcaggatccaacaggtagaagccctcatcactagcgccaaggcgaagccaaacgattcgcagcgcgtcgttttacatcgcctgagtatcagcatctgtcactcgaacctgttcatcccgatctaccatcgctacgttactcggttcggaggctatacgcgtattctaaagcatatacggcgtctaggtgacattgctgctgtcgctttcctggaattagtggactaatcgacaacacaaccggttcatcgcgccattccaagatccacaatgtcgcaagaacctccaagccagtacgtgaagtcattacgcaggtacacaatcgcgggaagtcaggattgcaagatcgctcttgtcaggtcacaagatgatcttgccgttgcctcaaagggtctcaggtacgacggctctggtcacgcgtgcaagaagttcgcaaagaccgcgttagaaggaacggtgcagatcgatcgacaatccaaggacacctacctggtccagatccctactgcgacagatttcgtagcccgagttccacgattctccagactgctgtactccgagtatactggaaactccatcagaggctacgccagataccttcagaagactaccttcgtcgatcgacgaagagccgtatacacagtcctttcagactcatcagctgcgattcgggaaacaatccgagtccggcgtatccctacctcaggacgatcaagttcgctcatcatcctaccatacacgcatatcggtatcagaatcggagttttagtgtctcactggcacttctccaactcgtaccgaaaccctattctggccatgcatgtcgctgctcgctcaccgagaagcctgagtatctacttcgtttacggtctggtcgtttcggaaacttcaattatacactccgtccagacgaagtctacgtctatcccttgttacatcggcttccgaaccgtttcgggccgcctgcgaaaggctctattcccaatagaactgtacggtcaaacgttcgttcagtcagaagtactcgcagtcgtctcacaacttagcttctacatcagcatcgttaggcagttcgaagataccaacgtgggagagggcattaacaagcctttcgagactttcctccgagaagtgacgttctacacgccaaagtaaacattacggaaccaagtattcccaggttcgccacctgcaagtatgatgaaggtcattttaaatgaatacgtgcaccctctgggcaacaccggtgacaagctcgaagtaaagccaggttatgcacagaacttcttgattatcaagaaggacgcggcgtcacataccttaccaagaattagaactatccagccagagccaatccagttcttccaaacgatatctcagaacggcgtcaagccgagtttaccaggattcaagttcaggcaccgttccttagagatctctcgaaagatcgatgacaccggcccactgttcggctctatcagtcgtcatcaaattctcgatcgggtgtatcggccatattcgtcgctgttcaagcagaacattctattatcgcggttacttacgcgaatatcgggacgcaagggtgtgtccctgcagctaattctggaggtcaatgcccgactccgtgttctggtcccggacaattaaccggtttcaacatcatcgcaggacgtactgccttcagctattatggcactggaaagtctgggcagcatcctgttcgttacacatacgacatcgaacgtgggccgtggtgacggaagcggcgcaggtaccacaaggggtcggggactcaagggctcctatgcacggacctcttatcgacagcttacccagttcgagggtggcccacacccattattcggacgcctgccggtattaggtgcagtcccgactgtctatctgtctacaggactcgtactcgtagtcaccgtaccggtatctgttactcgttcaacaggagtccgtcgatcttcgcttcatctactgtcttacatttcaccatctgcgttcgaggtaaaggtgctgctctcatctggaccgaagctgccacataccacttacagaccttaccctgctcgaaagcatcagccgttatcaagttccaggacaggtactacgaactaaacagcgttcgttacctacagtggtactacctttcgcgagacgtttcacgttcgataccacaccgaagacatctggtacaggagagcaaacttctaccaggaggtccaacttcctggtctacagctcattctcacaatcccgtacgcatctacggttccgtactaccgttattcacacctggttcgagacaaggcaccgtctatacagattctgcaaagaccggatccgtttccgagcagttacgcaaattcgtcacttctcctggcagaatgcattc

SEQ ID NO: 19 - DNA, 9932 bp, synthetic construct
  misc_feature 1..9932: note = seqHMM5002
  source 1..9932: mol_type = other DNA
gaatgctctcggtcgacttatccgatatatcccagaaccactcaggtacctgcgtcaagttcgcaactttacagaaagctccggcagagttccgaacagctcatcacaacaacgtattcggtcaggcggtacgcttatctgggtattacaaagcgttcgcagcttcggtctggaaagctttcccatatcaaggcgttcctgtcgtaccgttacaagcggattactgcatcacctgtcgttcgaacagtccacacacaacggtttcgtctcgcaaataatgtaccgaaagattaagatcggcgatagcgtcggtgttatctatggaaagcagaagggactcgagggtcacgtccactcagttctccggattcgataccacgtgatcgtcgaaggtgttttcagggacaagaagaagactaaggcaagactgcttatccaatcaggcggtccatcagaccagggagaacgtccgattcatacctccaatgttaagtctccgctgtactggcatcatttcaagcatccagttttcaagcgtgctctcgagcgatattcaaagaaccggcgcaatcaaggacagggcccagacatctaatctcttactcgtccgattctgtccactggacagcaattactaatgatctgcctgatttcctcgctcccgatcgtattccacctcaacagggtcaagcaagccttcgacagaggccaaggtgtgtgcgttactcagctcattccagaaggatacaagaagcgcgtccagcaattccgaggaacggtaatctatcaatccgatcgtggtcgcagaggcaatttccgggtggttaagtccagtcgcggcccaggcgtcgaacgtacgttccgtatctacgatctggtcattgaaggtattattgtggtcggaacgggcatcgtgcctcgtgcgacactcagctatttaagacgagtcagaggcaaggtcgacaagataaagcaatccttataaacacaggtcttctcaagccgtactattcggacgagttcagagatgatggcacgatcagcacgcgaactccgggtggttacaggcatctcgtcaagaatcacttccagtttgactgtacggatcagtgatcttatctcgagttcgcagaccgtctatctggttgagacgtcgttcgacctggcctccgcctacgtcttcgtatcgcagcttattgatccaggtatcagtcctgtatcagtcctaccactgcttctcgcgagaggcttcatccgaagtaccctggagtactccacgatcctcacacttcacccgccactcggattcattcgtgatttcagcctgagacgttcgtaccgaatccgaagtctgattcttcagctgttcgagccttaaactgccaacgacttcgattcaccttacgatacggcctatactatggtcgagtacttctacggatacccgctgacggacggcccaggtcagacgctcggccctattcttcgccgtgtcctcttaggtccaattgcaggttctgcgatctcgaggactctaattcgcccacaagaaatagaattcctcaatcgagcaggagtgcctgaagatgtgaactatatcattaggaacttgaagagcttggttcggcatattacttcatcgaagtcagccggtatctcgctggtacgtttcgatttattcgacggtcggagggctcaacgcagctggtattcaagacaagacgtcgaagtccgtttcagccctcacccaattaatcatttattacgtcgggaaactttggatattagcctgatcgtttactgtggcccgggctaccaccctttcggatccacatacaatcatctgcgcgcaactttcggcattacagtggatgcacgattcacccctgttagcttcgtgcactatacggttcattacgaattctcccaaggagcttctccggaagatgcactgtacctggatatccgaacttcctatcgccgaaggacatatcctgctttgtactgtgcgtcaccgtccctggaacagatcctgtcgggatatcatacacgagagcgcacgtacagatcctatacgcctactattcgagccactacggtcaaccgagagcaaattcagtcgaacagacaagacatcaccgaccttgatttgtcatcgcgctcgctgaattgcctgcgatccttcgtcataccaatcctgcacgaactggtgtctgcaggatacgccgaactaataccaaccggcaacttgggcgacaagtcagcctgggaaatctcgttccgtctcactgtacgtttcctggcgttaatcgtatcataacagcaggtcatacgtactctgcaaggaagtctcttccctgcaatgttcgacgatttcttacctgcgactgtgagttccggccgaggtggagtcggttctcgcttaccaaggatcgaacgatattcgacaaacggtggaccgccgggcggtctaggtggccctggcggttcggtgattcgaggtatctgcgcagttacttcgcatctttctgttcaatcgcaactcaggtcagcatacgcaacaccgggcagcgaaggtcctcaagaagagccagtaggtcgtcgcagaacatcagagccgatcatagtcccgcctggccgactagttacagcttctgcgcactatcataccgacaacagggtttcttcagcacgttcacgccattatacaggtcagggcggctacagaggagatggtaacaggtcattcaagaagctggaagaccctcttccgctgtcacgcacttctggcagaggtactacgtcccaaggactgttcttaccattatcttacttggccgatgttggtctcgttggtctcgtacaagacggcaagagcgcactgttgctcacaagagctgtatcgacacgaacaattaagctatacgtcttcataacgcactacccgaccctgggctcaacctgcggagaaccttatactccgtcctctcaagctgatattccgggcttaatccatctcagacacacgggatcaggcctgggtgtcaagttcttgacccatatcaagattcgagagagtctgcaagtactgatcgagagtcttcctgcattaccagacgtcagactatctctgcaccagaaggactcagtttcgttagtatcctatttacgtctcctgattccttcgatcgactgtactctggccagaaagtacgatttcaccgtcttccaacacgtacggtctcagctgcttctatcacggtcattacagcgaacattcctccgatcggctacatatcgcttccagttcaccctgttccatctggcggtactacaaccgctttccgattactaacctgttcactcctccgttcatacacgtccaaagttccaggaaatgcgaactgtagcgatcctgggcgccttcaactccggcaagagtactcttctcaacttattattacgtactgtaccgaggatcacatcttctcagcatctaacgaccctacaatctatccgaggtactcgaggtcatacgatacatcagaggattttcatcgatacaccgggcttatacagaaggaagcttcgatctgcggagctgctggcaaagtacatcatacgggcgctgatcacggtggatctgatccttttcgttgtcgcctacgctattcgtcaaccgagagatcactctctgacaactcgactgtctttacatcgcacttcgaggagactgtcgtcaccaacccatattcgcacttcgagtccactgttctcagactacactcctcgttacctacgagcatcctcgaagatacgaattgtgcagatttgcacagatctcggttccagcaattcacttacgcatcagacgaggagactcaagctacaacctttcatacgcaggaacccttcagatgctgtgtcggaccgtattctacatttcggtatcaaggaagttatccgtgaaaagattctgtcagccacccagaacgagatcccgtacgctgtccctgtgtccatcagatccgaaatctcgccagaggatttcggtatactcatcagatcgagcattagagtgctgcgcatctcacaaaagttaataatcatcggcaaggcaggtgatcacattaagtcaattggccctcatcgtcgcagcgtcctaattactcggatctgctcctacgtaattctcttcttaacagtgaagtaagaaggaccgttccttcttattcgcggacatcgattcacacctatgggacacccgaagactcagggacactctaagtcttcggacgcacgactttcgggttccagacgaggtcttactttagtgtccttcggtaagtacttcttagccattcatcgatctacctacattcgtcaagctcctattcaccgacgtatcgaggcgttacgacgggaggtccagttcatcggagacctgtggatacgcataacgtctctgccggtataccacctcaagcctgaattattccggatgggagacggcaagggtcgttcggaaacatggattacatcagttcatcagggcttcgtgttgttcgaattgtctggcgttggactcagaggcatcgacaacgctttggatcatgcatacgtcaagctgccaacataaactatcccaggtttcattacttccaagacggacctaccaggcatggtcctgttagtcgcggttagcggcggaccagacagtcaccagctcctgattcatctggcacgtctccgacttcaagacctgcatcgtactcaggccgcactggtcgatcatacataccggacagcatcctatatcccaagccgaatcgtctatcgttcactcggagtccattcaactgcaaccctcaacgattcctcacgaaagggatccttccgtccaatctgggtacgaaacggtgaaatcaccgcgcgctctcagcgttataacttcctcactactacgacaatcagggagaacctctcgtacattttgaccgcgcaccactgtgatgatgtaatcgaaacgattttgagacaactgcttcgcggtctatctacccagggcctgataggcttgcgcaatcctacgttcaactgcagaggagcaaatatctcgcgcccgctgctgatctcagaaaagctcgaaattccatctgcaggttcaacaaccagtttaaagcagtaccacgattacacgaattcatccgactcttactctcgtaatactattcgtcatcacttgctgccttaaaggtattcgtacgaactgcctcgttcgcctattcaagcctctatgattaatagcaagatactcaacggtgaagtcttcctgattttatcgatcggtggtacctcgctcattactctctacgttgaggccctggcaagcgccagcaatcctgtactggacttggttgtaatttcagttcgtacccatctgccggtagttaagattcttgattatggtaagtactcgtatgtatcctacaaggagactaagtaccggaagaagacgcagcctcaaatttgggtcaaggaagttgaactctctgttcacattcaaactcctgattattcagcaaagcgagctcactgtcgcaacttcctgacctacggttcgacggtgaagcctctagtacaacggtcaggccgattcaatcgccaacgatcgttatcgcactctgtgcttacgtacgtgtatcgtccaaacggtaccgtcatcatccagcatcaagagttcccacagagtccgttctcacagctaccgaacctgctgattccaagaggcccttaacacgaatcggatcctgtcttctgtactacacggtcgcttatcatgccggtcatcttattcactcttcggaggtccatcatcctgtcaggcgattcccagcatacctgcaacccgcagttcactcagttcatcctgctgcaccgtcatcaacacagccttatcccactggcgttccagtcaccttgccttcttacggtacaagcttcggtccgaacctgctccgactactcattcgacatactgttcgtgggcacaaagaacctctggtcgatattcgtctctccgcttgctaattccacaggtctctgctacgtgtctcagcgttggttgggtggcctactgaccaatactactaccataaccagcggcatttcaacgctgccggatctgttatcgctcacctggcacaagtcacagagacgctcgatcaagaaggaaagcgtcagagttaccatcgaaagagcgattttattctcctacctggctggaattgccaagctgcaagacgcaccgacgttcctcaccgtgttcgaccaagcacttgaagtatcagccgtgacagaggcgtatcgcctgtcgatcccggttgttgccggattcgatgttaatttcggcccgagacatgttgatgcgtccatcccaagtaatatccacgaacgcagttcttatacgttaatcgcgtatacatctggcacatcggttgcaacaatatccgcgtcctaatactctacagctggcttcccaacgaagtacgtccgtccattcatgttacacctgccgctgtcgaaggaagatccagtcatcgaacaacatcctaacccgaagtaccgttcgtcagactccttaaccgacgtactgagtttctcaaagctgcttcaatatcgaaccggtcatacgtcgagccagcttcagttcggcgacctcacgatatctaatctggaagtgtcaccggatgcgcaatcagccaccttcgtttacctggacggcaagcaattcctgtcaggacatggccgccttcatttgtcaggttatgatcatcaggtccatcgttccattacgccaatgcgcgctatagaatatcggattctgcagagatcgtcgtaatcgcgcaacatcagtcaggtctcatcaatctacgcacgatctatgtacactcgaagacaacagctgtacgatacggaccgcacttggagacgagtggatgcctcaagacgcatactgggccgccttgcttcgctcgttgcaatcgtattgtacggaaagcgaaaggtactctacctcccgggtctcgactctggcgatcaggttatcgtaattaatgctgacctggtaccactgtacggccataagaacacgcctaagcgctacacaggctattcgcagttcattggtcagcgttacacctcgctgctgttcaagctcgaattcctccaaccggagagttacctctccgttgccgtagttggagtgctcccgcctaccatactggccgcatcaaatcatctcgaactgcgtgtttaccaaggcactccgacaagagacatcgcgagtctcccgtacaatacctgggattaaacattctcgaacagttctgcgtcaatatcccaaggcgctcttatgagatcacaaaaggcggttcgttacctccgactccgtggtacattactccgcttcccttatttcgagctgctggagcatcgacgaatcagcaccacgatactaaagctactgcaccacttcgttcctgtagaattcttgattaccgaagcaaaggctatactcgtctcaaaccagcgccctgtgttcgtacgcctgttcaagagcacttctctacgctctttattcgttccaattgtcattccttacttacctcgttacggtggctatacccggattctcaagccaaggtcgcgcagaggcgatggagcttcctacgccgtcctggaactggtggactaatcacgcaagtacgacagcttcacaggctaccgaatacttcctatgaagcgacacttcgtatcaaggcctgtcaagaatcttcgtgatctaaccttcgcgaccttccaggattgcaagtcggcgctgtccctcgtacattcggacctgagcagcgccttcggcacgctgcgtattcgcggctacggttccgcgtacaagaaggcagtcccgattgcaaaggaaggctctgtgctactgtacaacgcactgctttctccgaagctggtggacatagattacgagaccgatttcgtcgccacagattcctctttcagggatctggtttatcgagagcgacgtattctcaagctgtccgaaggttctgttccaaagccgtcgttatatccagcacgagccatcaatcgaggaaacgaaccgttgattctgctcctcgcaactatatacgagaccatccaagtgcggcggatcctggcctcttacatttcctgcccagcttctatttacctttatctccacagtttcatacgtatcggtgtattagtattccgtcgcgatcctctctctacacgcgatctccatattcttgctatgcatgtggcggctcaatccccgcgttcactgatcaagctttcggttcaccggctgttagtatgccgttatttcagaatcatttcaccgccagcctatccgaagtcctcaccgttcgatattactcgaccgaacgtcgtcggacggttgttcaagacaagattcccaattgctctgcctgtccagactttcgtgatatccttcgttacggctgttgagcacatcctcttacgataccttcacgcagtactcactttctacatcggtatcgtgggcgaaggtatcctaaagagtatcgacaggttcatcctagaagtgccgtaccacgcattacaataacgacaacacgagtcgttacaccagaccagtcttaccacagatatgatgaaggttattttgagggaatccgtttcaacactgggcacgcatggtgacaccaacgaagttaagaacggctacgcatacaacttcctcatcccgaagtctcaagcgtacgcctatacgcagatcacaatcggacatcacccagaatctgtccgattcctcaacgcaagactctcccagtacacaacatcagccattctgccactgtacgcaagtcgaacgagactactgcgcatttctgtcaagacgggagaccctggtgtcctcttcggaaacattcatccgattcgaattctcgacgtagtgagaacgaacggttcgatcctgtctaagcaaccgatttacctgcaaaggaactggctcagcttccgcggagaggaggacgtttacctgtcgttactgctggaggtgtcagcgggtttgttcgtgacggttattctggtctaatcacgtcaatcctctcgacaatacgagattcagacgcgcattatgactttatcctcgctacaatctgtcccagaaagcccttccgacagacaatctgtcggacgcggaccaggttcaggcctcggtcacacgcatggcacgggcaagaagggtcaggctgctcgcgcaagagaaccttctccaagatacttcgaaggcggtcactgcccgttagattcccgcctgcctacgcagggctccgccgattcgtcttcttacgctatatactcggtggctgtgtctccgagcaagttcctacgctatttcagagctggagtgcggcaagctccactcaagaagctgtatcaaatttctgctacgccagtcccagtaaaggtgttaaagtacttacctacacctgcaaccggttctggtatcgtttacagacaataccctacccagcacctgtctggcacagttatattcgacttcagcacgtaaaacgaagcgtcggcaatttactgttcaactcacccgcattactgtacctgtccttctgtcaagagggtacaagtcggtcctacttcgcaaactcagcaaagggtttctcacgaagacccatccgtcacatatctggtatcctgtcagacgaagcagaggttcgaagcgatttcaaggtctactcgacagaggtcctccacttatccgtacttcacaagcgtcagtcctacactccgtcactacagatacctatctcagctcactcgggtatgcattc

SEQ ID NO: 20 - DNA, 9932 bp, synthetic construct
  misc_feature 1..9932: note = seqHMM5003
  source 1..9932: mol_type = other DNA
gaatgcacaccttcgcatcaagacctgcgaactacagataccaccttacagctggattccaagaccgggaaatctggaatccttcggttcttaccggacaatcgagctcaaagaaccgcagtcaactcttacatcgggaggacatcagtcttacacggctacacgtttacagcagacatcctggtccttcgatacgcctatctgctgttcaaatcgcacgtcgcatcacatcgagagtcgtcactttcaactacggagtcctcaacctgtccaaactatgcactataagattaagagcggagacagagtgacagtgatccctggcaagtccaagggctccttcggatacgtgagcttcgttacaaagggatctggaacggtgattgtggaaggcgtgcggaattctaagaagcgggaaaagtatccaactacggagacacatctgggtcttcaccgtctcaaggaaaggcctatccctgttagtaacgttgctggccttcggtacacctgtcacacaagcatctcagttactggccgcatccacgttctgtccagcaagtcacggaatctcggacgaactggtcagttcatataatccaagtattacaccttccgccaatctgtcaagatcgtccctatgaaggaacagattcctcgattgatccgacatcttcggatacgcagaataccgagccttttcagcgccggttacagggtaactgtacaacaggtcatttcggaaggtcacgtatcccgttaccaaattttcgtcggtcgtgttatctctgccacccttcaaggcgaattcagccctgctcaagtaaccaagtacgcatatggcccgggcgtagaacgtatcttcagctggacacgtactgcaattcatacaatcggcgtctcgttcactggcatcgtagagcgtgcaggtctcacctatcttcgcgttacaacaggcaagttctctaagattaagggttcatcgtaactatcgtaccggcttcaagatcgatcgcgtattcctcgcattatgatggcggctgtataccgaaacacgcgtgtacatcaatcgatcactgcgaatatccttcgcctgctccagtataccattgacgacggtacattcctctgtccacctgttcatatagtggaggattcagaggatctgctttccgcgcttgtcttcgtggctacgttaagcgattatacaaggtcggctatacaggttcgaagccttccaagtgccattggattcattcagtacagattgctgcggtacgcttcactgagagctcatccgactctgaacttctcgcctgatgcgagtttgtgtacaggagaacggatcgaagctctgattcacgcattgcacaatcggtaacgcacagatacaggacacttcccttacgatacggcctatactatggttgagtacttctacggatacccgctgaccgacggcccaggtcagacgctcggcccgattcttcgccgtgtcctcttaggtcctattgcaggttctgcgatctcgaggaccctaattcgcccacaagaaatagaatttctcaatcgagcaggagtgcctgaagacgtgaactatatcattaggaacttgaaaagcttggttcggcatattacttcaagtaagtcagccggtatctcgctggtacggttcgatttattcgacggtcggagggcacaacgcagctggtattcaagacaagatgtcgaagtccgtttcagccctcacccgattaatcatttattacgtcgggaaacattggatattagcctgatcgtttactgcggcccgggctaccaccctttcggaagcacatacaatcatctgcgcgcaacttttggcattacagtggatgcacgattcactcctgttagcttcgtgcactatacggtccattacgaattctcccaaggagcttccccggaagatgcactgtacctggatatacgaacttcctatcgccgaaggacataccctgctttgtactgtgcgtcaccgtcgctggaacagatcctgtcgggatatcacacacgagagcgcacgtacagatcctacacgcctactattcgagccactacggtgaaccgagagcaaattcagtcgaaccgacaagacatcaccgaccttgatttgtcttcgcgctcgctgaattgcctgcgatcgttcgtcataccaatcctgcacgaactcgtgtctgcaggatacgccgaactaattccaaccggcaacttgggcgacaagtctgcctgggaaatctcgttccgtctcacggtacgtttcctggcgttaatcgtaagctaacagcaggtcatacgtactctgcagggaagtctcttccctgcaatgttcgatgatttcttacctgcgactgtgagtagcggccgaggtggagtcggttctcgcctcccaaggatcgaacgatattcgacaaatggtggaccgccgggcggtctaggtgggcctggcggttcggtgattcgaggtatttgcgcagttacttcgcatctttctgtgcaatcgcaactcaggtcagcatacgccacaccgggcagcgaaggtcctcaagaggagccagtaggtcgtcgcagaacatccgagccgatcatagtcccgcctggccggctagttacagcttctgcgcactatcacaccgacaacagggtttcttcagcaagatcacgccattatacaggtcagggcggatacagaggagatggtaacaggtcatttaagaagctggaagaccctcttccgctatcacgcacttctggcagaggtactacttcccaaggactgttcttaccattatcgtacttggccgatgttggtctcgttggcctcgtacaagacggcaagagcgcactcttgctcacaagagctgtatcgacaagaacaattaagctatacgtcttcataacccactacccgaccctgggctcaacctgtggagaaccttatactccgtcctctcaggctgatattccgggcttaatccatcttagacacacgggatcaggcctgggtgtgaagttcttgacccatatcaagattagagagagtctgcaagtactgatcgagtcacttcctgcattaccagacgtcagactctctctgcaccagaaggactcagtttctttagtatcctatttacgtctcctgatcccttcgatcgactgtactctggcccgaaagtacgatttcaccgtcttccaacatgtacggtctcagctgcttctatcacgctcattacagcgaacattcctccgatccgctacatatcgcttccagttcaccttgttccatctggcggtactacaaccgctatccgattactaacctgttcactccagcgttcatacacgtccaaagttccaggcaatgcgaactgtagcgatcctgggcgcctttaactccggcaagagtactcttctcaacttattattacgtactgtaccgcggatcacatcttctcagcatctaacgaccctacaatctatccgaggtactcgcggtcatacgatacatcagaggattttcatcgatacaccgggcttataccgaaggaagcttcgatctgcggagctgctggcaaagtacatcatacgggcgctaatcacggtggatctgatccttttcgttgtcgcctacgctattcgtcaacccagagatcactctctgacaactcgactgtctttacatcgcacttcgaggcgtctgtcgtcaccaacccatattcgcacttcgagtccactgttctcagactatactcctcgttacctacgagcatcctcgaagatacgaattgtgcagatttgtacagatctcggttccagcaattcacttacgcatcagacgaggagactcaaactacaacctttcatacgcaggaacccttcagatgctgtgtcggaccgtatcctacatttcggtatcaaggaagttatccgtgaaaagattctgtcagccacgcagaacgagatcccgtacgctgtccctgtgtccatcagatccgaaatctccccagaggatttcggtatactcatcagatcgagcattagagtgctgcgcatatcacaaaagttaataatcatcggcaaggcaggtgatcacattaagtcaataggccctcatcgtcgcagcgtcctaattactcggatctgctcctacgtaatactcttcttaacagtgaagtaagaaggaccgttccttcttattcgcggacaccgattcacacctatgggacacccgaagactcagggacactctaagtcttctgacgcacgactttcgggttccagacgaggtcttactttagtgtccttcggcaagtacttcttagccattcatcgatctacctacattcgtcaagctcctatacaccgacgtatcgaggcgttacgacgggaggtccagttcatcggagacctttggatacgcataacgtctctgccggtataccacctcaagcctgaattatttcggatgggagacggcaagggtcgttcggaaacatggattacatcagttcaccagggcttcgtgttgttcgaattgtctggcgttggactcagaggcatcgataacgctttggatcatgcatacgtcaagctgccaacataaactatcccaggattcattacttccaagacggacctaccaggcatggtcctgttagtcgcggtgagcggcggaccagacagtcaccagctcctgattcatctggcacgtctccgtcttcaagacctgcatcgtactcaggccgcactggtcgatcatacataccgaacagcatcctatatcccaagccgaatcgtctatcgttcactcggagtccactcaactgcaaccctcaacgattcctcacgaaagggatccttccgtccaatttgggtacgaaacggtgaaatcaccgcgcgctctcagcgttataacttcctaactactacgacaatcagggagaacctctcgtacattttgaccgcgcaccattgtgatgatgtaatcgaaacgattttgagacaactgcttcgcggtctaagcacccagggcctgataggcttgcgcaatcctacgttcaactgcagaggagccaatatctcgcgcccgctgctgatctcagaaaagctcgaaattccatctgcgggttcaacaaccagtttaaagcagtaccacgattacacgaattcatccgattcttactctcgtaatactattcgtcatcacttgctgccttaaaggtatagttacgaactgcctcgttcgcctattcaagcctctatgattaatagcaagatactcaacggtgaagtcttcctgattttatcgatcggtggtacctcgctcattactctctacgtcgaggccctggcaagcgccagcaatcctgtactggacttggttgtaatttcagttcgtacccatctgccggtagttaagattcttgattatggtaagtacagctatgtatcctacaaggagactaagtaccggaagaagacgcagcctcaaatttgggtcaaggaagttgaactctctgttcacattcaaactcctgattatagcgcaaagcgagctcactgtcgcaacttcctgacctacggttcgacggtgaagcctctagtacaacggtcaggccgattcaatcgccaacgatcgttatcgctttctgtgcttacgtacgtgtatcgtccaaacggtaccgtcatcatccagcatcaagagttcccacagagtccgttctcacagctaccgaacctgctgattcctagaggcccttaacacgaatcggatcctgtcttctgtactacacggtcgcttatcatgccggtcatcttattcactcttcggaggtccatcatcctgtcaggagattcccagcatacctgcaacccgcagttcactcagttcatcctgctgcaccgtcatcaacacagccttatcccactggcgttccagtcaccttgccttctgacggtacaagcttcggtccgaacctgctccgactactcattcgacatactgttcgtgggcacaaagaacctctggtcgatattcgtctctccgcttgctaactccacaggtctctgctacgtgtctcagcgttggttgggtggcctactgaccaatactactaccataaccagcggcatttcaacgctgccggatctgttatccctcacctggcacaagtcacagagacgctcgatcaagaaggaaagcgtcagagttaccatcgaaagagcgattttattctcctacctggctggaattgccaaactgcaagacgcaccgacgttcctcaccgtgttcgaccaagcacttgaagtatcagccgtgacagaggcgtatcgcctgtcgatcccggttgttgccggatttgatgttaatttcggcccgagacatgttgatgcgtccatcccaagtaatatccacgaacgcagttcttatacgttaatcgcgtatacatctggcacatcggtcgcaacaatatccgcgtcctaatactctacagctggcttcccaacgaagtacgtccgtccattcatgttacacctgccgctgtcgaaggaagatccagtcatagaacaacatcctaacccgaagtaccgttcgtcagactccttaaccgacgtactgagtttctcaaagctgcttcaatatcgaaccggtcatacgtcgagccaacttcagttcggcgacctcacgatatctaatctggaagtgtcaccggatgcgcaatcagccaccttcgtttacctggacggcaagcaattcctgtcaggacacggccgccttcatttgtcaggttatgatcatcaggtccatcgttccattacgccaatgcgcgctatagaatatcggattctgcagagatcgtcgtaatcgcgaaacatcagtcaggtctcatcaatctacgcacgatctatgtacactcgaagacaacagctgtacgatacggaccgcacttggagacgagtggatgcctcaagacgcatactgggccgccttgcttcgctcgttgcaatcgtattgtacggaaagcgaaaggtactctacctcccgggtctcgactctggcgatcaggttatcgtaattaatgctgatctggtaccactgtacggccataagaacacgcctaagcgctacacaggctattcgcagttcattggtcagcgttacacctcgctgctgttcaagctcgaattcctccaaccggagagttacctctccgttgccgtagttggagtgctcccgcctaccatactggccgcatcaaatcatctcgaactgcgtgtttaccaaggtactccgacaagagacatcgcgagtctcccgtacaatacctgggattaaacattctcgaacagttctgcgtcaatatcccaaggcgctcttatgagatcacaaaaggcggttcgttacctccgactccgtggtacattactccgcttcccttatttcgagctgctggagcatcgacgaatcagcaccacgatactaaagttgctgcaccacttcgttcctgtagaattcttgattaccgaagcaaaggctatactcgtctcaaaccagcgccctgtgttcgtacgcctgttcaagagcacttctctacgctctttattcgttccaattgtcattccttacttacctcgttacggtggctatacccggattctcaagccaaggtcgcgcagaggcgatggagcgtcctacgccgtcctggaactggtggactaatcacgcaagtacgacagcttcacaggctaccgaatacttcctatgaagcgacacttcgtatcaaggcctgtcaagaatcttcgtgatctaaccttcgcgaccttccaggattgcaagtcggcgctgtccctcgtacattcggacctgagcagcgccttcggcacgctgcgaattcgcggctacggttccgcgtacaagaaggcagtcccgattgcaaaggaaggctctgtgctactgtacaacgcactgctttctccgaagctggtggacatagattacgagaccgatttcgtcgccacagattcctctttcagggatctggtttatcgagagcgacgtattctcaagctgtccgaaggttctgttccaaaaccgtcgttatatccagcacgagccatcaatcgaggaaacgaaccgttgattctgctcctcgcaactatatacgagaccatccaagtgcggcggatcctggcctcttacatttcctgcccagcttctatttacctttatctccacagtttcatacgtatcggtgtattagtattccgtcgcgatcctctctctacacgcgacctccatattcttgctatgcatgtggcggctcaatccccgcgttcactgatcaagcgttcggttcaccggctgttagtatgccgttatttcagaatcatttcaccgccagcctatccgaagtcctcaccgttcgatattactcgaccgaacgtcgtcggacggttgttcaagacaagattcccaattgctctgcctgtccaaactttcgtgatatccttcgttacggctgttgagcacatcctcttacgataccttcacgcagtactcactttctacatcggtatcgtgggcgaaggtatcctaaagagtatcgacaggttcatcctagaagtgccgtaccacgcattacaataacgacaacacgagtcgttacactgccgaagaatctcaccacgtatgatgaaggtcatcctgtctgaaatcgtacagggtctgggttcaacgggagatcgggtcgaagtcaagtacggctatgcgtacaatttcttaattcagaagtcttctgccccagcgactacgttactggcaattccttctcaacgtcgaagctcgtacacaacattccagcgtcaatctctcgcatcaagcatcgctgttatcaacgcgtcgggaatacaacagccgaatttgtcgattgacgataaggaccgggactcaggacacctattcggcagcatccgtcgagcagagatcttcgatcgagtctatcggttccatacaccattatggaagggaattatttcgttacagacatcgatacgagacaccaacggtgcatatccagtgattctgaagctttcgtacgaggtgactgccggtctgagagttctcgtacagcgctcttaatacttcgcatccgttcagatcctctcgtactctggaacctacatgcgcctgcgtcacctgtacgacaactcgctggattctcacatcaggagctcagtgggccgtggagagggttcgggcttcggtaagacgcgtggctcaggccgaaagggacaaatcgcccgtatcctcgataccatcgaactcaagttcgagggcggtggactaccgctgccgtcacgattaccggccgatggcggaatcggtcaaatccctctcagaactgcttacgtgttcgttgctgtcgattccacggattctggtccatacaccatcgtacacaagggagttctccgacatctgccttctattgagcaaccttcatcagacgtaaaggtactgccatcaactgtaccttcaagaatccggcttctcacgacttcctcgtatcagtcagagtcttacggacgtcagacaatctgcggaagtcaatacacgtaagtaccacacgaagtcccactaagcttctctggctgcgaactgttcttactgcagagacttcgccaaaggttcctgcaagcacaatcgacaaacgatcgcacttcttacgaccgtcgaaccagatccctttatcacagccttccttcttcgactacggaaggagcggtatattccaggaactgttcctatccactcgccagagcgaatatctcgcaggtattctcaattcggttctcgcgagcagatactacccgaagcttactacaaggcagcattc

SEQ ID NO: 21 - DNA, 9932 bp, synthetic construct
  misc_feature 1..9932: note = seqHMM6001
  source 1..9932: mol_type = other DNA
gaatgccgtcacctgtcaagtcgcagaccatctgcactcggccagtcggacagtctttccgcaacccgaatcaaccggtcgagcgaggaacgtccgatcgcaacgacaacgaatcggcttcccaccggcaccatccaacagcgagtacgtatccgcacgagtccagctggccacgcaactaccagatacctcgagcgagatacccgctcacgcgcaccgaatcagtctacgaagggagtcctcgtcgccactccacctgctgggaaaggccactcttatgactgtcaagatcaagactggcgatactgtaaacgtgatcgcaggcaagtccaagggccagttcggctacgttccgacagtctcggactaccgtctcagcgtgatcgtggagggcgtgtcgagcactaagaaggtactcaagattcggactgcgctcagtctgcacggttccggtatcttcccagaatcaccgatccctgtcagcaatgtgagtacagcaaggaactccgacctacgacttcggccggtcggaattcgcatcggaccggtcatctggaagagccggcgccacaacttctacggctcggcgatctaaaggtcacacgccctcagaacatcgccagagttcgctcaaccaatgatcccacgcattttacacctgagcttcccaggaggtaccaggctatcggaggcgtacttcctccgaggcgccacagtcatcgtaatcgccggtatcgtcgagggttacccgaatagaatccaaggattcccgggcgtcgttattggtcctgagaagcatggcggcaagctacgcagacctgtacagaagggaagtattggttacggcgtggaacgccgcttcttccctccattcgtttcgatccgacggattatcgtggctaccaacggcactgtcactcgagccgtcctgcactatcttcggcacgtacacggcaaggtccctaagatcaaggcatcggtctaaacgaatccggtatcccaaagcgtcgacctgctcggaccttcaatgatggcggtcaactgccgccatcggcgcgtgctcgccagaatccctggcctaatcgcttcatcgctgatctgtccgatcgaggaccagtctcagctacctctcggtgtgctgcgggtggaggagtcgcgtgacttggtaccagcccaagtcttcgtgtaccggctgatcgacccagtattcggcacgagcgatgtcatcgacttgaccgtcgccgatggtttcattaccgaacgattgcttcgtcgaggacacctctccgtcgcgccgcggctgactttccaaagggaccaatcgctgtcggcggaaccgcgtatcttctctttgatttcgctacttaccgcaacctaagcgtcctatctacagtccgtcgaacgctcgactcccattccgatgcgttcgtcgttctgcatctcaccgctgccaccaggtctgggcaccaccctgggcgagttactgcgtcgtgttctgcttcacgtaatcgcaggaaccgcgatcagagcgtcagatatacacactcgccggatcgagttccgacctggcagtggtgtgggagaggacgtgcgcaacatcatccgaaacctgaagtacctagccctctgtatcgctcagccgtcgagaaggactgttcgcggccaggatacacaaccgaagccgctccttctagctcgggacgagtcacgcatactggtcagtgtggaagtctccgcgcggacgattcgcattaattcactcgactccgtacacctgcttcctatcatcttggctgtcccgggaggactcggataccgtacccgccaaaccggtttcctcggacagagttcgactcgggacatttcagtcgacgcctcgttctcgccggtccgcatagtgcggtacacggtggtccaacctgtcgtccctggaagtctacgccctgataagctgtcattgctcatcgcgacgcatacgtcgacaggcaacgttcgtgcgctgagccctgcgccaatctggctcctctacgctctgaaggctcaggaggaccggctactggtccactacgcatcaccgtccaagcacccacctcgcatcaccgttcctgtacggacattcgcagtcatccgacgcatcgttacgttggatctgagcctacgtactggtaactgcctcctcaacaacgtcatcggacctctggttgaactggtgggcggtttaccggcaccgctcactacccatcctaatttgggccgtaagtcgcgtccggagattagaagcgtactcgcaccgacgaccctgttcctcggtacgagttaatcaccacaggcgtctgccgagactctgctcacgaactctaccatgttcccggactccacgtctggcagggtcaccaatggcggtggcggtgctggaacacgaggctgtcggcaagagatatacgcggacgcgggcggcccgacgggcggcacgggcggccagggcggacaggtcagaggctaccgggccaatcgtactatcgccctcggtccacgaaagcgttcgccggtcacgtacgcgctgcgaggcactctcggcacacgacgcggatcggatggtatcggttctggacgaacggacattgtcgtcccgtctggtgagtccgtgcgacgtactcaccgttctcgtccgtactcgttaccgggcgaaaggtaccctacgtacgcttcgggacagggcggccaggccggcttaggcaaccaagcgttcaccactgcagtcgagggaatcccgaagaggtcttcgcctggatcgacgataccgcaggaggccctgatcctctgcctttcccgccttgccgatgtgggcctggtcggcttcgagtctcggggtaagagctggctgttgacacgtctatcactctgcagcctggacatcttccggtacggattcccaaccatacacccgggcctgggtatctgccagccttcggacgacttacgaacgccgccggccgacatcccgggtcttattgacgattcgtacccaggtgctggcctgggttgcaggttcctgtatcacatcgcacgtcgacgttatctgggcagactgatctcacttcgggccaacacgcctatacctcttcggctgtcgcgaagacctcaggtcacctgcctcttaccttacgcctacagcctgacagctgtcccggagtctatcctgccagataagctggactcgttcgaggcttcagagcacgatccactcggcctccatatccgaccgtctcaacagggtctcacagcctggccacaacaggaccctgctcaagcactccgtattccgggctacccatcgcacactgcccacacataaactatccctcgcttctcgcagcgcaggacttcaggcggatatatgcactgcgtcgcgatcttgggcaccaccaacctgggcaagagcaccctgctgaacaggttgtccacctaccatccgtatatcgtctcccgaccttgctcgacaacctatcaccaaatcgagggcctgcgcgagctgcgttcggcgcaagaaattttcattgacacgcctggcttgtcgaagccaaaggagtaccggtctacactactcaggaagcctatcccagcggcactacacggtgtggaccttatcctgttcgtggtgcaagttcacggccgttcagttacggacttcccgctcctggcgacactcgacctccatacagcggctactctcctcgtcgcaacgctcagtctaccgatcatcgcgtacgaagcggcgtccacaaggcagcttcctccacaaagctaccgtccaagcaccatcgttgctatcaccacttcgaccatcgaccggctataccgcgcgagggtatcgaacaagggcctcctcgaaggttacctcggtcctgtaccgcaagacagtgtacgtgacgagtctacgggcttcttcattcttgagctgattcgggaaaagatacttggtcgactcacggaggagattccatacattgtgggagtccagatcgcaaggacgtaccagtcgactttcaccggctctctgatcccgtatcgcatccctgtctaccgctgcagtcaaaagcttataatcatcggcgttcgtggagaacgaatcaagggcataggcgcgtcgtcacgacttcagctttccagtccggcggaccagcttgtcactctgtctctgcaagtcaagtaagtccacctggactggtcagcagtctctacgaggagagcttcgatgcgacctccgaagagggtatacccaggtaagacgctggtccgcaagtcggagggcgacttcccttccgatacccacgtcctcttcggcagatatcgcctgtacgttcgactgtccggagcaattgtcctcatcgccatcaccttccctggaaacgcgctggctcgacctgtaagctcgagtggtggcctgtggctgagaatctgcgagctggaaactgcaagctcgaagccatccggacgccgcatgggccagggcaagggcccgacagaacgctggaggccaatcgtggcccagggcaccgtccttttcgagctcgctggcgtcctttcggccaagctctacccagcgctgtacgtcgccacagcaaagttgccgcactaagtctgcagctgccaaggcactctcgagctacgctctggttacatggtcctgttggtggcggtcagcggtggtaccgactccgagacactgctccctctgctggcacatacctggcagaagcaccttatcgcccagccggcagcgggtgtcgatcatacacaccgcgttcactcgagggcacgtcctacctcggtggctcacacgaagcgcaccgctcctgaagcggtatctgcaagcagtctgtcaggtcgacacgctggcggcaagaaggactcccaacaggagccggcggcccgcgagggacgctaccagtcactgcttcgcaggtccaaccgcaggagttccgctcaaattttgaccgcacatcacgtcgacgacagaatcgaaaccatactcttccgtttgctccgtggccgacctcatcacggcctggcaggcctgctcgctgctacggagagctctgctatcggtcaaatcttccgtccgctgctggtcatctggaagacggaaatctcgttacctgcggtcgtcaagcagctctcacaggtctgcgactctaccaacggacctacgtactacaagcgcaacgtaatccgctcgacgcttctgccgtaattcagagtcgcgttcctcaggaactcgcggctgtatccttcaatgattaatacgccaatcacggttcgagaggtgtcgggaatcgccacccagggcttacttcagtccatcgcagaacgtcgagaggccctggttcaagcgtgctgcaagacactcgatctggtcaccatctcgtcagattcccgaaggcctgtcgttaagatcttggattacggcaagtacacgtacggtacctctaagggctccaagcgggtaaagaagagtcaaacgaggattaccgtcaaggaagtcagcctgatctacgttattcctactccggacggtacgtctaagactgtcaagctcacgaagttcctcatcggaggcggtcacgtgaagtctcgcgtgcttcaccgcggtcgcgttccgacggcttcccaactcactcgaagcgtgcttagggtcgtgctcagctggtccgaagtacacaaggcgagctgtcgtcactctgcccagctggtactgtactgctcccggtctctgctgcagccgcctccgcgataaacaatctgccgcagtcaggttcagcgtcctaccttcacgtcgatgcaggtcgcacttgtttctcttagacagcaggcctcctataccggttcgacgtccatccgctacgacccgatcgccaaggacttcatctgccgacagcgtttctgcctcagacgaatcttactcaggatcggccgctacctgctgcgacatacggagcaattcgtggcgccgcctactcctggcaacattccgatcctgttcgtcggcacgaagttacgcgtacggagtactgtgctgttccacgccgccgcacactcgtatcggtatgtcgtccgacgctggcttggtggagaactcgtaaacgccgatacgattgcacggataatccgagctcttagctctcttccgagacgccctgtaccacacgtcctcacccattcaggaaagaaggagagcttctcgtactgggtaccgacctcattcctctcggacgtcctcttcggcatcggtaccctttacgaggccccgagactgctgggtgtggtcgacctcgttcacgaaccgctagcggtgaaggaagcgtgtccattgcagattcctgtggtcgcctgcgaggaccgcaactccgcgccgacaagtgtagaccagaacatcccgatcaacgaggcagcgttcaattcggcgacgctgtcgtcccactacagcgcacgcttcgtctcgagctccgtctgcacgtaaggacactgcggaaagatcgttctcagagcggcttccggtccgatgctaccgctcagactgcctgcacaggacgtcacgcgtacaaggcgatacaatagcatctatcgccagagcgacggcatcaccgatgtcttgtccttcccatgcagtaccgagcgtttcgcaccactggcttctccaacgcagcctgtcggtgacctcaacatcagccaggtctcagtgggagtcgcagcgtcacctcgtacgactctccgactgccgggaaggagtcaactgcctcgtcacggctccctgcacttgcgcggctacgaccatcgatccacaactacagccgcgggaatggttcacaccgagcgcataatcctcctaccgctcccttaacatctgcagactcgaacctgctctcattcacgggctcaccgcatgcgacgcatcaacccttcacgttccactcggtcgcgacggtgggaggtagtcgatgccaccgcgatcggacttggtcgtctcgctgagcaagtcgctgtacgcctgggcggtaagcgcaagcactcatatactccagtcaacgacgctggcgatcgagtgatcgtgatcaacgcgtcgggagtcaccctctgtggccgtaagaccgcgttcaagccttatgaccaagcttcctctggaaccggtctcagtattacgccacgtcgtacgagcctgcgatccgcaggaatcctatcctacctgtgccaagcggtcccgggcatgctcccgcctgtcactctgaaggcgcgtccactcgacagcctgcgcgtctaccgaggccgactcccgagcttcagtgcacggtccccgtatacgtacgaaggataacctcttcgctgcagcgccggaatttctcgagacaggactgccatgggcactggcaagaggtaccgcttcgacaccgaacggagcacgttgctgcgtgctacaaggcatacgctcctcagtcggtctccgattggcacgaccgtcgctaagacgtcagcctccgtcagacgtgtcgagacactgatcacactcgccaaggcccaataccgcagctccgagcgaattgtgcgaaccaccctggacactcaggcaggacagcacttcctcttctcagcgattccactacgataccaccctcgccagggaggctacacgcgtatcctgaagctgtccgctcgtaagggcgacgctgcccgcaaggcctctttggagctggtcgattaaagctgcgaaccggcaagatctcgaccatcccacgatcggttcatggtacgggacttccagcgaactcgcgtgaagccactgcgccgcagaacctgggcgtctacccgggactgcaagctcgcactggacagtcgcagactggatttgacccacgcgagtcgtcctctgcggatcggcggcactcgctcagcggagaagaagctctccgacgctgctgaggaaggaagcgtgaacgaggttcgagaggtttcggcctatcgactggtgagcatcccgggtactactgatttcgtcgcaccgagggaccgtttcactgtcctattactccgaatcgccgagctccgtcgactggacacgttcagattcccagcacgtccgctctccacggatacgggatccatacctgcacacgtcgtcctgccgcaaactccagcgggagtacgggaatccatccgggtcagacggatcgctggaagcttacagtactctcaggctctcatcgtaccgtacaagcatctatcaagtcgcatcggcgtgctggtcctgcacgtcggctacttactgctctggaccgcaacctctctggccatgcatgtggcggcgctcgctcctccttcactgctaccggcggaggtacgaactgctactgtcgcggcaaacacgatcatcgcttccgcatactggatacggcctggcgtaccgatcctcatccagcacgtactcgtgagcggccgtctcatcaagctcaagcctgacatttacctgacgtcgcaacagttcgtgttcgaatccggcgactacgtccattcggtcctcttacgcctaccaaggcacgtgcatcacttcactggccctctagtgggcgagggaattggtaagtgtcgcttcaccttcctggttgaggtcatcggaccgaactacgcctaacatcacgccctatccggactatctccgctgcaatccgcagttatgatgaaggtcatcctcttcgaactggtctcgcagctcggcgctcggggcgacggaccggaggtcaagctcggctacgcgaccaacttcctcatcggtaagcgtacagcgtacggttacaccacgcggtacatcgtccgggcggattacacatcagcgttcggcccagatcaggacgatccgcctcagaagagtccgtactgccgctacacagcaactggacggccattcctcggcatcttctgcaagacgctggaccctggaggattgttcggctccatccgctcacaccgtattagagattcggtcattacgcctacgctcaagctgggtaaggcacacatccgactcgttctcacgcggaaggtccctacgggcgcgacaccggtcacgctgtccttgccttacgaagtatgcgcgggactccgtgtgctagttcgcgtcaactaaccaagcccgtctcacagttccaaggtctggacagccacctcaatgacgctccctcctttgataccttccgctggactctcctgcgtaccacggaccgtcggacgcggcccaggctcgggtcagggccacacccacggcgaaggaccaaagggatgggaggcccgcagacgtcatccgcgaacaatcagattcgagggcggcgtcacacctcttagcgttcggctgccgaggtcgggccctggatcgggttccacgcctacttctgtaccggtcgcagtccgtccagtcacgtctggctacaggtacagcgcagaggtcttcgcacctcgcctaccaacgaatcgacgcatcgagaacatcctgctcccagtcaaggtgctcaccgccagctactcgaaggccactgctggacggtatccactgggcacactggcgaatcgtcagtcgccgtcgagattccgctgggcctactccgactaaaccacgagctggacttcactggaacgtactgtcacacaccggccaagctcaagcgcgagcttacgccttcaatacgagccgggcagttcacccgacctcattctggcaacccaatacgcctcgcctcagaggcgtcgtatcgtcagcaggattcaggcccaatcgagctgcccactccgagagcactcctacagagttcctggacgcttcctcgagctcacccggtacaacacctcacagaggcgcactacacgacttcgcgccagcactagcattc

SEQ ID NO: 22 - DNA, 9932 bp, synthetic construct
  misc_feature 1..9932: note = seqHMM04
  source 1..9932: mol_type = other DNA
gaatgcgggcccatcgtatttcgtttccgttctattcgtcacagagccctggacgattacgaagtatccgacagtattctcgaaccctcagcgtctcgacaaagtacacacacgattcacacatcgggtaccacctcaacagaactatctcggagcaacagaacctacgggtctgtttccgagttacttatccacgacagccttactgcgctcaaagtcaggtcatctgtatccctcatccgattcccaactcgacgtatccgagtcggaaaccttcatgctgtacaagatcaagttaggcgaccaggtaatcgtgattgatggcaagaagaagggcctctacggttcggtgaccttcgtccgattcgctcggatatacgtgatcgtggaaggtgtccaacatcgaaagaagcatcagaagccgggagagtacaactggattccaggctctcactgcagtttcgaatcgcctatttcaacgagcaacgtgatcacggactaccttccaatccgtacgatccagtacgtcctatcgcgtacactcttcttcagcgacaagacccgtgtcacggaacatcaaggctcaattatttaactcttcccgatacctgcgactcaacgtattactctcgcaggaatgactctcgagatcctgtacctgttcgtctacagccctgcaatacgatcgcttcaggttttcgaacacggccaagacgtgtctgttgctggtcctattgttgagggccgtatacggcggacccagcgattcgagggttgcgtcatcactcatcgtctcttcggcgcgactacaagacttcaggtaagaaagatccacttaggaaccggagtggaacgtaccttcaatctcagctcagacaagatttcgacaattactgtggatccacgaggcatcgtggctcgagcccgtttagcatatctcagagacaatccaggcaagctcgcaaagatcaagctatcgcagtaacgattaccgaatccagactcggacacatctatcggcaagtctatgatggccggacctcttcggtcgtctcgtgtgcaagcaaacattcctgcagccatttcactcgttctgactcgcttaattggtgatcacccaagacgtatcagcagtgtgcacagagttgaattcagcggagatctgcaatacgcgagtgtcttcgtcttactgctgcgcgatatcgcatcaactcagtctgtcgtgggtttcttgcgtcgcgcacatggattcatttcagcttaccttaggagactggcgcagttatacagaaacccaatcctgcgtttccacggcgacccgagtttagaggcagttctgcgcatccaactgctgatcggttacctgtcagcaacgtaaagaatcatacgaggacctcgtttactacatcgttcaatttcaatgttatcgttcttcattcaaggaccgttgtcaaagggacttggtatcactttaggaaaggaacttagaagagttttgttataccaaattattggattcgcgattgtattcatcagaatctatacgtatatacctgaattcgaattacgatctggcgtcaatgaagatgtatctgtaataatagttaatcttaagttcttagaatcttacgatacttatatacgagaatcatcgttccaaagttctgttcacatattattacagatcaagagtgcttacgttacctacaagaattatattattgttgaagttctggcactacaaagagttatcatattattgagattccatccaaggttacaaatacatcttattgtattatcaggatacggatatgcttatatcgatacagttatttacaagttcatatcgactcgaataatcatcgtagatgctttcttcttacctgtaacagttgttacctatttcgtagaaagattataccatcatatcgtacaaattcaagattcgcttatattattaattttcacatcgtatatcgaaagacaattcgtagcattatatctggctatacagtatctaactcttcaattaatcggattcacaaagaagcatcgtatttcaaacacgtattacagattcctcttacagaatatcgatatcttcgagttattccaaatcgacagtatcattatctcagttttagatcttagctaccgtcgtcataattgtctacaacgtatattcatttatattttatacgaattagttttatctggaatattcgaacttctacaagaaagtaatcttggctacaagagcattactgaaattatacaattcttactattacatactctctaccttggaaatctataattacactgttattctttctctatcagaagatctttatcttctatgttcatcgatgagtattaccctactgtttattcaggattaggcggttctggatatcgatctcgtattctagaactctatcatatatcaggcggacctcgtggtggtctgggtggagttggcggacacgttttacgtattcaagatttccaaatacgattccttaacaacgtacgtattcatttacacgaatatgcagatattggccaaagtggtacgatacaaatcgatataggttcaaagaattattcgtattcgatatcagttcctcatggcgaattcgtgaagatatacaacagcttcacagaagaattccctgtattatccgatattatacagatactatcgaatcttggcggtgaatcgggtttaggcaatcaacgattcctcatatattcaacacggattccaatcatactacgaaacggcatatcatatcctgtacagatattattattaaacttattcaagttagcagatgttggacttgttggcttccgaatattaggtaagagttcacttttagtatctatattcagaacacattcgttcatcacatcttacgctttctatacattcagacctcagcttggatatacgagctcagtattatatatcaagaaggctgttgctgatattcctggcttaattaatattacttcagacggtgaaggattaggttacgagttcttataccatatctattatcgcttccaattaagacaacttattttattcaagttcactcagtcaattcaaacaagtttcgatttcaagtcttattatccatacttaaaggactaccaagaatctcttgatttactattcatccaggtcaagcatttcaagcgagatttcaaggaaatcattcaagtacagaatacgtacatattcatacagaagtctctacgattcaagggaaattacttacagtctatatacgatctattccattacaagcaaatcaagggatacagtatacacatatattaattcgaaatcaagagttcttatcaatatacagtttcgttacagatgttccttgttgcaatacttggattatctaacgacggtaagtctacattacttaattatttaaagtcaaatcagttctctatctctagcaagttccttatcaccaccttcgaccttattcacggatactacagaaattatttacgacaattcattttcatcgatacccctggtttatatatatcgaagcatatcgaatacaagcttttaaacaagtatatctcgatagcgttactgttagttgatcttatacttttcgtagtaaagctattcctggatttatcacaggattccaagttatacctgtacctttattcagagtatacttatcagtccttacatttacaagtcaagaagcttatctatacgaacgaactttatcagttacagagtattcaattcaaggtcaagtcactttatcgaatagtattcataattactattatacgggtattatcatcagacattatcttcaaggttcatattcagttaattacttctatacgagaagatcctttagattgtgtttctgattcatacaaggacttcctgattatagaatatattcgtgaaaagattttacgattacgacatatcgaaattccttacgaagttgatgtttacatagaagatcagaagtaccagaagttcgagaattattacatttcttaccgtatcattgtatatagaagaagtcaaaagtccatcatcattggcattactggacagaagattaagtacattggatcacaagtaaggttcactctcagtacagaaatttcatcacgagttcatcttacattgttagtaaagtaattatatccatcgaagcattatagggaaccaagtcgggatcttatgcaagtaccgaagaaggtcactcgactcaagacgaacatcaccagtatatccggtgctcactgcaccttcggaaaggtgaccttcggtccttacaggttaaaggccagtctacaagcttacattcaaacctgggaaatttcgcctcaaggaagtgctctttcacggacggtaggaaccaccggttggctgtggaatagaatcgaattccaggctcagctccgagaaaagccattctctccgcgaatgggtgctggcaagggcagtctcgaactgtggtcagccaatgtgatcagaggcttcgtccttttcgagttatatggcgtgcggactcaagaagcgagctcagccctatcccaagcagaagcaaagctgccgcgttaaagagcgatctctacgttccagcaactcctctgcatctggctcatggtcctgctcgtagccgtcagtggcggaattgacagccgtaccctgctgcagacgcttaagtcagccttcaacagcagtcctggctatttccaggccgccccggtggatcacgcgagccgtattcagagtagtctgggtatctacggtgtctccgcatacgttctctggctttcgccaatactacagaagtcgcagttctctggaccaactgtccagttacgtctcaagccaggcttcgcatgcccggcccgccatcgacgctacatcagcctgaagtcagctgccaaggatttctgtcatctcaccatcctgacggcgcaccaccaggatgatggcatcgaaaccattctgctctctctgcagcgcggcctttcaggtatcggcctgcatggactgcagctattcgagcgatccaagaagtcgagcaacattctccgccctctcctgccttatcgaaagatcgagattgagttcgaggacatcaagggttctctgcaaagtatccgtgatagaactaaccgaactgcccattaccaccgcaacggaatccgcccttcactgttaccgtaattatcagcaaccgccattccttctcgctacaggtactctcaaatgatcaacacggatatctactaccgagaagtgctatcaattaacttcagaggcgttcacgtcaacatcgccgcagaaatcgaagcattgcaactggcaacagctttacctttagatttggtgagaatcagtagcctactacgtatacctgttgagaagatcctggattacggaaagtaccagtatatctcgactaagctgtcgaagcgcaagaagaagtaccagaattccattccggtcaaggaagtatctttgttcgtcaggatccatttcgacgatactgtcgacaagcagatccatcgattcttcttcctgcgcgtcggatatcaagtgaagatacgggttatcttatccggccgttcgtcgtatcaacggcagctgtcgatttctgttttgacgttcgtccgttacggttcggaagtcatacaatccgacaccgtttcggtctcaggactgtcattccatcatcgcagaaggctcctggctccgacgtacgaataaatccttacggacgacaccttccgtataccaccaagcagtttcatgtcggtcgaattgttactgctcacagaagcgttccgataccacggctcaaccaagttcgacggactaccggcacaacatacgttcattaatcctcgacgctccaccagtcttcgaatttgtttaacatctacgctgttctccctgtcgtattcagttctatccgtgagggaatccctatacgccaagctaccgattttattcgttggcaccaagttcatcgcctgtctcgcggtatcatcctccgcatcccaaagattcccaggatacgtactaccgcgctggctgggtggcactctgtcaaatagaacgaccatcccgcttacaatcccacaactattacgtctgttcacggattacgctcctcactcaagactcgcttcacagaagaaggaaatttcggccagcttccgatacggctatcctctgttcagcatcttgccgggaatttattcattagacactcagccgcaagaactgcgcgtgcttgaccaagtcccggaaaaggatgcagtcattgaagctggttacctgttaatcccggtagttgcgaattccgaccacaacaaggcgccgaccgatgtagattgtttcatcccgccaaattatcacgcgttcggtccaaggagtctgaagaagtccttccgaacttacgacgttccggatcaaacgattctgtaattaccaaccgaaatccacccaatcgacctcacgaccgctcggatggtccacctgaagctggagcctggagactgtcctggcgcgtacgcgttaaacccacgataccgcgactacgaccgagcgaccgacgtcctgtcgttcttcgcgcagctggtaccacgcatcgcacctgcacttccgcagccactcggaggcgacctgcgcatcagcgcgtatcgggtgatctggacggcctcacgggtccaggcctaccatcaccctcgctcggaggcactccgatcgcatggcaacctccacctggccggctacgaccacccgaagctcacggttcgcgcagcgatgcttctccctgaacagtcaatcctgactcctacgcgataagcgacgagggtcatccgctatccgagcagttcgccgcagctcatgagtcgatctggatcgatacaccctggtcgactgcgccagtggcggattgtggacgccgtccaggtaccgctgggacgcctcgccgttctagtggcctaccggctctcgggcaagtccaaggctggctactacccgatcggcgacccaggcgacgacgtgatcgtgatcaatgccagtcgggtgcagctgctcggcgccaagttcgagtctaagacttatggtaccggcagcaaccgcctcggtccagcctacgtcggtaccgtcaggacgctgaggcggacagcttacgcgcaccctctgcgaagtgccgtcaggggcatgctaccgcaccgcgatctcccgtcgaactcatccgccagcctgcgagtctaccgtggcccgagtcgaagcaaggcggcgccgaagccgtcccgctaccatcagtaagtcctcgccgaacgtcctcctgtacggcctatacacgccgtcatgcgagcgtccaagagccaccggacccatacctcccgcccaaccctgctgcgcgcgtacgaccgactcctgctgctactcctcggcatcagcaccaccgctgtcaagaggcgagaacctccggcaccggtggaacgactgatcaccgccgcgaaggtcctggcgggcagatctgcgcgcaaggtgtccacaatcctgctccgcggttacaccctcagcgtactgttctcgagtatcgagcacggatatggtctccgggctggcggttacacccggatcctcaagctggcttctcgcccgggtgacttagcgctcggtgcgccgctcgaactggtcgattaagacgtcaggagcgaagtcggctcccaaaccgcgcctaagtcgatgtaccgagcttccggaacctgcgaggtaaagccgctgcgctcacacacgggagccggctcacgggactgcaagcgtgcgctgagctcaccgttcggtgatctgtcgatcgcgtgcggcgcactccgcagcaagggcgcgttcacggccgttaagaagaggcgcgtcacagcgggagagggcagggtcctcacgcgtcactgccctgcggaggctattctggtggcgatcgtccaggcgaccgacttcgtagccactaccgactggttcctacgcctgcggatccacgcggaatccacctcgcatctcactggcaggcctctcgcagccgctgtactctccgtatcgggcatcagcgctggtacgggctggcaactgcgatcgctctccgccgagcactcagagccgatcccagtgcgccggatcgaggctcgcaccgtctcgagcatcggcgaaatcattccttacgctcacaccctcagccggatcggcgtgctggtgtcacggctggccagcgataccactggcctcggaacgcgcctggcgatgcatgtggccgcccgtaccccacgtcaactgaccctacttcgcgtgcatccaatctgcgtggcctcaggaccgcatatccggagccgatcgaagcctcgcctcgcactgccagcaggcattgcgtacgagcctgtttctggccgcttgccgaagcgcaaccgacgtatcagactgctgggacaggcgttcgtggtcgcggaaaccagggttgtgggcggtcgactgttcaagcctccggccaaggtgcgtctgttccgtcgctggactgtgggcgagggcatccataaggcagcacgcctcttcccgaaggaagtggccctgcaggaaggcctataagcgagacctgcgacgtcttccgcgtatcacaacccatcgtcaatgatgaaggttattctgctcgagcaggtgaagaagctgggtaccgtcggtgacctactcgaggttaagcacggctacgcggttaacttcctgattctaaagagcgtagcctcagatcgtacagactctataattgcttattcgccgaagcgacagagttcaggactccaacacaacgtcaaccaactcaggacaacggtcaagccttacaggaataccggattcataccgttatcgattgaatctaagtacaatgaccgcggttcgctgttcggctcgatcactgccaattatattctcgatgtcgttagctctccaaagccttcattgttaaagtcctggattgtcctggtcaccactctcgtatactcgtcaggccttaccgctgtgacgctggaactggagagtgaggtaatagccaacctgactgtggtcgtcactactggctaatcttaccaagcgcatttccgtctcgatctccaactcgaattcatgtacctgcctatcttggaaccaacgtcaagccggatactgtacgcttcagtagtgggtcgcggtcgaggcagtggcctcggtctcactaatggcaccggacataagggatctgtagcgcgcgatccacgattcttcgtcgacaacttcgaaggcggctgcaggcctttgttccatcgccttcctgctacaggccgttactctggtcattcaccaagattcgagaccgtgaccgtgtgcgtactcctacacgcctatataccttgtacacgagtgtgcctggacgaactaacggtttatacgtccataacaactactgtcgagagggttaaggtgctcacggagctgcaacttacgttccagcatctgcatcgagagagcatcactcgcggaatctattctgtccgaaaccggttcaatccagtctgccacgagtaaacacagtacactccacgttcacttccagctttcaacgataccgacgcactattcgtccgattcagcacaacgacactttcactaccgctcaacacgttcagcaaacagggtacgcgttacttcagccctatacttcacgtactcctcaggagtccatcgagacacttcgtatctacagtatcgcccttcagagccctcagagattccgaaatatcgttacgcgatcgttcgacgcctccgatcaattcagattacttaccgaggttcggcagcattc

SEQ ID NO: 23 - DNA, 9998 bp, synthetic construct
  misc_feature 1..9998: note = seqRANDOM01
  source 1..9998: mol_type = other DNA
gaatgcgtcaccgctgttatccaagctcatacgtctctgtacaaggcctgggtactcttcagcgttcacctgcagtacatttcgcccgagtcttccatactcgatcacgagttcctctttcagggcctctcaacaagatcgattaccactgtccacatccctttcgggatcaagtcaacgagctactcactcgttcagagatcacccacaacaacctgtaccgtccatatcgagcagtactcgatccagaagacgcaatctgctccatttcccatacgtcgttcagagtatcccggattctgcagtatcaggaatcctctccgcacattattcgggtacagaggtctcttacgagaggacgtcaacacaaacccggattcaacgaacatccagagcttcaggtaccagactactcggaacattctcagtcatccgggtatcgtcaagaagcactgtcgagcatcttacaactcgaccctccgtttcctacatactgcacccaagagttctcaatcgcctaccatacgatcttccctacgactgcgatctgtcaacagcaaccaagcgttctatcgtcacgctaccagcatttaccaggttccacctggtatcaagaaccggcactatcgtttcacgagtacagggtacacttcacgaagcccttcagggatattactcgtcgttcagtctcgcacaaagtcggctactcatcagttacggaatctgttcgtcccaaacctcgcaaagcagttcggatcacataccgatatcagggtccactaccttcgaacgtcatcctggatcctcaaatcgtacgcaacccgtatcatcgtacggaaagacggaagtaccagttctcccgtttctacatctctcggaacaaggtcctgcacaactcaggtaccttatcgttccatcgtcattctggcagagtcagcagtccaagcaagactacgtactcagaagacacagaacgcctgcaaacgcattacgagcgaacaagaagatcgaaatattctcattcagttatatctactgtctgtctatacgttacatttacgaatttcaaagaattcgtacagtacgatatcagaatttacaagcttatttatatcagagatcaaggtacttcagaatttcatacaagaatatacctgtttacaagtaccagtttatcaatcttatcgatattacgtcatatcatctgtcaaagaacattcaagatatcaagaatcctttatacatcgactattcaagaagcatcaaacaagaattcaaatacatactgccaaagattatcactatctgttatttcgatatacaagagaagaagtcaatatactatcgtatcagtttcttatatctcagtcattacagtttacgattatatcgaacacttattcgtactgtttatcaaagtcgatcttatacatcagtttatacgcaattattcacgaaagcattattatcgatcaacattatcgaagattatctgtacacagattacaagtacatattccatacgttatatcaagatcttcaaacggatatttatcgtattacgatatctgttactatcgattcaagaagtatacagatattacaaacgaattcagaagattacgtcttacatactgtttacaaactgtatacaacgatacattacgatcatacgaaatttacgttatctatacgatctttcgtatttacgttactgtatctcgttatattatcttcgagatattacttcaacaacgtttatcgcaaatatttacgagtttatattcgcaaggttatctatcgattattattatcgtccttatttcgatcaggaatctttatcaaagcatttatctgctgttattatcatcgttacgtatatacagtttcacaaagtcttcgtatatatacatcggatatcattcagaagtattacgtattcgtcttatttatcgacaagtctatacaaatcaaacgtatactgtccaatttattacgtactgttacaatacgatttcagacaattctatcaatttcgtatcgtcaaatattcaatctggtacaaagttactgttattcttcaagacatttacagattcaagatatcactctatacgaaagaatacaccaaatcaagaatttcaagcattattcaagacttcgtatatctgtttcaaacatcttacagaaacagtacatattctcagtatatcgatcttattcaaacgattcatacagtcaaagtcaaattacgacaaatacagtacaaagacaagatttcaacaagctttacagtatatactttacgagaatcgtatttcagtttcacattacagttattatacgattcagttcatctacgatatatcgttccaaatatacttcagtacagtacaatttctatcgttacgaatattctgtacatatacgatacgtttattcatcacgaagtcatattattcgtttattcaacgtatctattcgttactgtacaagttatcacagtatttacaattcgagtatatcatcgactctatattacgaatatacaagtacgatatcagtcattatccgtttatatactacgaaacaagatatcaactacgttatcgtatacatacattacgttatacagcttacagatcagtttcagaaatatattcgaatttcaataccgtacgaacttatcagcatttatatatcgaatatttcaccaagaagcgtatcaatacagaaattatcagcatatttcagatcatttcgttacaagtacgtatttacaaagattcaatcgagaatttcgtatatacgacttcaattatttcagtataccatcagtatacttcaagacgactttattattacacagttcattcgaaagtattcattcaggtcatttatatattcagatcagaggtatcgtatattcgtcaacaatattatattacgacgatcattcaagacttacagaatactgtttatatatcagacaggtttaccttatcaggaatcaaagattattacttcagactacgaatatactatccagagttacattatatacatacggttacctatatacgtttatctctgtcattatacaaatacgttacagatctctatttcaagtatcgaacatacttacaagaaagttcacaaagattcttcaattcaaggtatcgaaatacacagatacatacgttatattacgtttccaaactatcgatttacacagaaattcattactgtatcgacaaatatttcgtactaccagtattacatttcgacatatacagtattattccaagttcaagtattccagaatcagaagttcttattatatcggaattatccagtttatcactcgatattacagttattaccagaatttcaacgatatattcgagagaagttcatatattacagtattcgaaaccaagattcttcatttctgcatttattcgatcaatatatcagctatacaagatctctgtacttattccacaagatttatatcgattatatctgtcgatacaactattcgaaagagcatattacttacaaagaactgttctctatcaaagaatacgttcatcaattcaagaagaatcgatcaaatcttacagtattacagcttattacgctattatcggtttatatcctattacgaagaatttctctcgtatatcagaaatttacatctggattatacttcgttatcacgaacttattcaagtatttcgaaatcacatacacgccctgctctattctcgaccgctatcctgtatatactcacgccaggtacaaagagcctgtcgcgttcaagattcaagtcaggtcacttctcgacaccgacagtcacagattcaacaatcacgacgtcagactccgacactgctgtcaaattcgttacctgctcacggaaactgtcgggactttcgctattcagtatcagcgccatctggaagtccaggaagtccttctgtatcttcactgtcctcctcgaaaccagctcgtcttcagtccattctacacagctaccgatccatacgtctgtccgctgttacaagagcttccacacgcatttaccctatacgcctgcatacctatcgtcacccagctcagaatttcaacgtacgaggtcctcatctgtccacagacctcgatttaccatcagccttccagagtatcccgctcacttcaggaattcacgtactgcatacgccatactgcagcgtacgacaagtattcgtcaggagttccagttcaccagaacgttcgactacaaggtctcacgcacaggaatcatacgaggtttccgcgaactttctgcaagcgttcacagcatattccacagccgccaacaatacttccctcagttactcgactcatcactgcgagcaagttctcactgctactgtacgtttccattccgatcggtcaacctcagcaagtacaacccaagtctcaacggtttcgatccgacactaccgacagatacagatcccttatcgaacgtcagctggacacaagtctcgtctactgtcgttacaaggacggagacagtctttcgaggtactcgcttcgtatctacgaagcaggcaccttatcgtactgtctcaggagttcactgtacggagtccagatcttcgcagactattacgctggttccactgtcgctacgacaatcaagggtttacaatcgccacttcctcagccatacgagcaacgaactaccatactcgcgttcaatcgcccaatccagatctcctacagagatcacacgaacacttcaccggtacagcttacagccaaagctgttccaacacagttacacccggatctcaacttccgaacgaattccgcacaatcaacaagggcgacaccttctgccattcttcaggctttccatatctctgcgccaaacgtacgcgtattcatacgcgatcaatacatcgcccagggatacgcagaatactgtttcccagcaacaagtctcggtcccgaatctgcacattcgtatacgctcagtcaaggaggtcggaaagagtaccacaccagttatcagccgactactatccgaccatacgaagagttccagtccagatcacggtacatctgttcgaaccatcggtcatcgtacgagctacagcttacacctctcgaactcttcgtccacaactgtcaagggaaagataccgcaacgttcactcgacgaggaatacttcgacaacaggatctggacgaagggtcaacgagaaatcaacgcagcacttctcaggttacagcgtacacacaccgttcatctcagaacgtcctgtccaagatctcatcatcgacctcgatcacgcatcaatccgaccagatctgtatactactgccgagggttaccgttcagccaggattatcatacgtttctcccgcctcaactcaacgggaaaccgtcattatctcgattcgagcctacctccgattccaagcccaatcaaagcatccaactgcccaatcaccacgtcgttctgcgaattactcgaacgacaaggattcgaaggctcagcgattccgattacagacactcaaaggcagctaccttcggactgctctttcaagccagagaatcaccactgtacaggcgatacacagctcaaacagcgaaattccagcgcttatcggagtcagtacggtattccggaaaggtactatccgaaggaggtctacggttacatcgaccattcgtcacagaacgtcttacggactcgaaagctacgaagatcgcacaagtccgaaagtcgcagaaacttctcagccttacgcaagcgaagggatcttctgcttcagttcaggtacaggagaggacctgtttctaccttccaagatccggtctttccaacctcatccgccatatactgggcatatacgacggaatacccgtacacgtcagtcaacactcagaagatacccggaatcgtctcgaagagagccaaacatcgtccacattccacaactgcaactgggatcctgtacgcaaatcgctctacgtctttcacagccaaggaactcgcttactacggcaagtttcggacattccatcgacaaagccctcattcgtctccgaagatcacctgttcaagcaatccacagcaagcgatatcggaacggagttacgtctctcagtaccagtccaatcagtcgagacactgttatccggttcgaagacgggagacaagtttcaggacaagctactgcgataatcgccacgcgtacctggcctcccagctgggccgatctatcacggaacgcgctcgagcagacccgctggctcgactacagactgctcggatcggaagggccgggtccagtccaggtcattacctgggtctccggagctcgctcggctaccactggactgtcagcacgcctacgggcatcggccatcaggctaccgcaagcgtacgcgccaatccgggatacgggtccgttacctcccgtctcaagcgcgctccaccgtaccgtcgcgcaaaccagactcggaaatcccgcgctaccctcccgctgcgacaggtctgtctctggaatcacggcaggcctgctgcaccggcacatcacgacactcagctgggcacgaggctgcatccgcccgagacaatcgctcgatcactgggtcgccgaacgccgcctgcacgattcacatcccaggactggactgcggcccgctactcgcgcaatcgtaccgatctgtcagggccctggacgctccaaggcgctcacttccaacaggctcacacgccggatcggagccagctcgagtcagtacccgagcgactcccgttcccatcccgcgttcgagagaggtacactcccgcgggactcacagcggtccacatcccaggatctccacccgagtccacggaagtccgcgacagtcgggagtcaccaagtccagtcccgcacgaccgactccctctcacgccaaaggtcgacgctggcgacgagtacccgcgtacatcgggtaccgttctcccgtcggagccctacgcggtttacggtccgtcttccgagtctcgcacggccgaccagtcaaggtccgagagcaagctcggaccctcgactcgcgagccacacgacagctctgcatcacgcgaccctctccacgggcgatctgctcgacacgacaaagctgcggcacctcgcctgcgaaacgggcggttacgatcaacggcgaggtcagcacccgaccctgcgcgaactttctctgccgagcccatccctcgcaagtccgctgccggttatcctcttcgaccgcacgtcggcactcactgcaggccgctacacgctttcctctccgccagctgcagccacaccgacactgcagcgtacgtctcagcccgagcctcatcaggacgggtcctcagcgaactaccgcgcgatcagctcttccgaggcccggatcgcgaacgtacacccaggctccacatcgaggacgacggctctcgcaccttcgctgggagtccatatcggcccacgtcgcacttccctcgaagggcgatccggcatacccgtcgggattcgaccctgtctccgctctcgagcacgctcacggcatccaggtcagaccctcctggcacgaagtacgccggcttcctcacacgtctaccgggaccgatcgagcatcggcagcccacttccggtcagactccgcgacaccgactctcggaagcgcactgccagaggatcccacaccgacgtcaccgcctatcgccgtacggagtacggcgtacccgttccactcgccgtcatcggacgatctccggtcggagcaaggcctcgtttcccaggccattcgcccacacgtcgggacttcacccggttccactcgcaaggccgtacgaggctggctcacagcccatactcgaggagcccagagtcggacctcgccgaaccacactcgtcagtccggaaccgcgacgttcgtcgtccacctggtcaggtacggactctcgcctcggatcagacggctccgtactcctcggatcccgctacggctgcctacgtcagacgcgtcttcacccgcaggtacgtcccggagctacctcagggcaccagacactccacgtcgcaccatccggagtcttcagcgcggaagctgggagagaggctccgacagtcccaaccatccgcacaggctccctgctttcgaccggagcccgttcaatcccgtcctcaccagcgcaaggccatacccggtcccaactggtcgaccagccactggaagcccactggcttccacccactgcgcgttcctcccactgctcgaggcacaaggtctgcgaacggacgctcgtccggacagcgtcgcactatcgagacgcgtctgccgcaagaggctggtcaggccgtatcaggtccagccgttcgagcccaacctaccgggcctcaacgctcaacgcaccagctccgcagtcccatcctcggactcacgaacaccgcctgcactggcgcgtcatccgtactcgagagccgagaggatcggcgatcagcggacgagtctgctcccaggaccagagagctgcgaggacttcgcaggactcgagcgccctcagatacctgccagagcccttcgcctcagtccggtacggctacgactcgtcgaccgtacggtcccgaagggtctccgatcagctccgctgcagggtcagagaggtcagcctcacgcctcgaatccggaccaccgctcaagcgactccgcatccatcccgcagtacgccatccgcagcagtcagcgcactacgttcgacgcgctgtcgacgtccacgccactaccgacatcgcactcgagcaggttcgcgcacggcagctactacctgcgctcttctcagcgcggagcctgctcctggattctcccaggcctggtaccacctctgcgcgccaagggtatcacggaggctctggcttccgagggacgggactctccatcagcgtcgctacagcgcatcacgccgcttatacagcacggagtcacccatcagtacactgggagtatctattcggaggctgtctacgcactcgtttcctcaatctggaatcaacgacgtcgaagcagttcaccttccttcgtcagaaattccacgcgaacactacgggtcttacaggtcccactttcaatccaaggacgtatcgctacgcactctatacggtccttcgatactcctactacaagccgaactcacctaccaaacctggcagtcaacattactcagcctactgctctcatccactacggagatcacacttcagttcccaaaggcctacatcaactgcgaacgcctgtcaagtatccactctacgatctcgctatcggacttacgagacccattcggtttcaacagagtctgctccgattcgacagttccatatccgagaatctggccttcggttctcagtcagtcaaagtactcagccgtacagatcagacgagcgatcactcatacggtttcacgagaaaccgactacgagagtcagctatctgctgcaaagtcgagtttcacaggcccaaccagatcgaaattcgcaaacggtccaatcagaacggcgactctacatccattctggactacgaggtatcaagccctcggatcaactgtcaaacctcgacaactcagacttcgggactacgtcgaaatcacagacatctccgcaaacgttacggcaaccaagccttactaccagcttctcactggtatctgggaaagacctggctatcgatccaacctcatcgttcagtacctcaaacgagacggtaccgaagttacgttctgcagttcacgttccaagtcctcgattcgcaccatcagtcacgatatacccacaggttcgtacgtacgagttcccagtacctatacagaggtcgttcgcctatatctggcactcgaagagtcttacacctcggaagcagatctctaccaacacgttcaccgttatcggaggtcagcgtagcattc